European Patent Specification EP 3 585 164 B1, published December 27, 2023. Title: NON-HUMAN ANIMALS COMPRISING A HUMANIZED TRKB LOCUS. Applicant: Regeneron Pharmaceuticals, Inc. The sequence listing filed with the application follows.

SEQUENCE LISTING (125 sequences)

SEQ ID NO: 1 - protein, 821 aa, Mus musculus
  MISC_FEATURE (1)..(31): Signal Peptide
  MISC_FEATURE (32)..(429): Extracellular Domain
  MISC_FEATURE (430)..(453): Transmembrane Domain
  MISC_FEATURE (454)..(821): Cytoplasmic Domain
MSPWLKWHGPAMARLWGLCLLVLGFWRASLACPTSCKCSSARIWCTEPSPGIVAFPRLEPNSVDPENITEILIANQKRLEIINEDDVEAYVGLRNLTIVDSGLKFVAYKAFLKNSNLRHINFTRNKLTSLSRRHFRHLDLSDLILTGNPFTCSCDIMWLKTLQETKSSPDTQDLYCLNESSKNMPLANLQIPNCGLPSARLAAPNLTVEEGKSVTLSCSVGGDPLPTLYWDVGNLVSKHMNETSHTQGSLRITNISSDDSGKQISCVAENLVGEDQDSVNLTVHFAPTITFLESPTSDHHWCIPFTVRGNPKPALQWFYNGAILNESKYICTKIHVTNHTEYHGCLQLDNPTHMNNGDYTLMAKNEYGKDERQISAHFMGRPGVDYETNPNYPEVLYEDWTTPTDIGDTTNKSNEIPSTDVADQSNREHLSVYAVVVIASVVGFCLLVMLLLLKLARHSKFGMKGPASVISNDDDSASPLHHISNGSNTPSSSEGGPDAVIIGMTKIPVIENPQYFGITNSQLKPDTFVQHIKRHNIVLKRELGEGAFGKVFLAECYNLCPEQDKILVAVKTLKDASDNARKDFHREAELLTNLQHEHIVKFYGVCVEGDPLIMVFEYMKHGDLNKFLRAHGPDAVLMAEGNPPTELTQSQMLHIAQQIAAGMVYLASQHFVHRDLATRNCLVGENLLVKIGDFGMSRDVYSTDYYRVGGHTMLPIRWMPPESIMYRKFTTESDVWSLGVVLWEIFTYGKQPWYQLSNNEVIECITQGRVLQRPRTCPQEVYELMLGCWQREPHTRKNIKSIHTLLQNLAKASPVYLDILG

SEQ ID NO: 2 - protein, 821 aa, Rattus norvegicus
  MISC_FEATURE (1)..(31): Signal Peptide
  MISC_FEATURE (32)..(429): Extracellular Domain
  MISC_FEATURE (430)..(453): Transmembrane Domain
  MISC_FEATURE (454)..(821): Cytoplasmic Domain
MSPWPRWHGPAMARLWGLCLLVLGFWRASLACPMSCKCSTTRIWCTEPSPGIVAFPRLEPNSIDPENITEILIANQKRLEIINEDDVEAYVGLKNLTIVDSGLKFVAYKAFLKNGNLRHINFTRNKLTSLSRRHFRHLDLSDLILTGNPFTCSCDIMWLKTLQETKSSPDTQDLYCLNESSKNTPLANLQIPNCGLPSARLAAPNLTVEEGKSVTISCSVGGDPLPTLYWDVGNLVSKHMNETSHTQGSLRITNISSDDSGKQISCVAENLVGEDQDSVNLTVHFAPTITFLESPTSDHHWCIPFTVRGNPKPALQWFYNGAILNESKYICTKIHVTNHTEYHGCLQLDNPTHMNNGDYTLMAKNEYGKDERQISAHFMGRPGVDYETNPNYPEVLYEDWTTPTDIGDTTNKSNEIPSTDVADQTNREHLSVYAVVVIASVVGFCLLVMLLLLKLARHSKFGMKGPASVISNDDDSASPLHHISNGSNTPSSSEGGPDAVIIGMTKIPVIENPQYFGITNSQLKPDTFVQHIKRHNIVLKRELGEGAFGKVFLAECYNLCPEQDKILVAVKTLKDASDNARKDFHREAELLTNLQHEHIVKFYGVCVEGDPLIMVFEYMKHGDLNKFLRAHGPDAVLMAEGNPPTELTQSQMLHIAQQIAAGMVYLASQHFVHRDLATRNCLVGENLLVKIGDFGMSRDVYSTDYYRVGGHTMLPIRWMPPESIMYRKFTTESDVWSLGVVLWEIFTYGKQPWYQLSNNEVIECITQGRVLQRPRTCPQEVYELMLGCWQREPHTRKNIKNIHTLLQNLAKASPVYLDILG

SEQ ID NO: 3 - protein, 838 aa, Homo sapiens
  MISC_FEATURE (1)..(31): Signal Peptide
  MISC_FEATURE (32)..(430): Extracellular Domain
  MISC_FEATURE (431)..(454): Transmembrane Domain
  MISC_FEATURE (455)..(838): Cytoplasmic Domain
MSSWIRWHGPAMARLWGFCWLVVGFWRAAFACPTSCKCSASRIWCSDPSPGIVAFPRLEPNSVDPENITEIFIANQKRLEIINEDDVEAYVGLRNLTIVDSGLKFVAHKAFLKNSNLQHINFTRNKLTSLSRKHFRHLDLSELILVGNPFTCSCDIMWIKTLQEAKSSPDTQDLYCLNESSKNIPLANLQIPNCGLPSANLAAPNLTVEEGKSITLSCSVAGDPVPNMYWDVGNLVSKHMNETSHTQGSLRITNISSDDSGKQISCVAENLVGEDQDSVNLTVHFAPTITFLESPTSDHHWCIPFTVKGNPKPALQWFYNGAILNESKYICTKIHVTNHTEYHGCLQLDNPTHMNNGDYTLIAKNEYGKDEKQISAHFMGWPGIDDGANPNYPDVIYEDYGTAANDIGDTTNRSNEIPSTDVTDKTGREHLSVYAVVVIASVVGFCLLVMLFLLKLARHSKFGMKDFSWFGFGKVKSRQGVGPASVISNDDDSASPLHHISNGSNTPSSSEGGPDAVIIGMTKIPVIENPQYFGITNSQLKPDTFVQHIKRHNIVLKRELGEGAFGKVFLAECYNLCPEQDKILVAVKTLKDASDNARKDFHREAELLTNLQHEHIVKFYGVCVEGDPLIMVFEYMKHGDLNKFLRAHGPDAVLMAEGNPPTELTQSQMLHIAQQIAAGMVYLASQHFVHRDLATRNCLVGENLLVKIGDFGMSRDVYSTDYYRVGGHTMLPIRWMPPESIMYRKFTTESDVWSLGVVLWEIFTYGKQPWYQLSNNEVIECITQGRVLQRPRTCPQEVYELMLGCWQREPHMRKNIKGIHTLLQNLAKASPVYLDILG

SEQ ID NO: 4 - protein, 822 aa, Artificial Sequence
  Synthetic
  MISC_FEATURE (1)..(31): Signal Peptide
  MISC_FEATURE (1)..(31): Mouse Sequence
  MISC_FEATURE (32)..(430): Extracellular Domain
  MISC_FEATURE (32)..(432): Human Sequence
  MISC_FEATURE (431)..(454): Transmembrane Domain
  MISC_FEATURE (433)..(822): Mouse Sequence
  MISC_FEATURE (455)..(822): Cytoplasmic Domain
MSPWLKWHGPAMARLWGLCLLVLGFWRASLACPTSCKCSASRIWCSDPSPGIVAFPRLEPNSVDPENITEIFIANQKRLEIINEDDVEAYVGLRNLTIVDSGLKFVAHKAFLKNSNLQHINFTRNKLTSLSRKHFRHLDLSELILVGNPFTCSCDIMWIKTLQEAKSSPDTQDLYCLNESSKNIPLANLQIPNCGLPSANLAAPNLTVEEGKSITLSCSVAGDPVPNMYWDVGNLVSKHMNETSHTQGSLRITNISSDDSGKQISCVAENLVGEDQDSVNLTVHFAPTITFLESPTSDHHWCIPFTVKGNPKPALQWFYNGAILNESKYICTKIHVTNHTEYHGCLQLDNPTHMNNGDYTLIAKNEYGKDEKQISAHFMGWPGIDDGANPNYPDVIYEDYGTAANDIGDTTNRSNEIPSTDVTDKTGREHLSVYAVVVIASVVGFCLLVMLLLLKLARHSKFGMKGPASVISNDDDSASPLHHISNGSNTPSSSEGGPDAVIIGMTKIPVIENPQYFGITNSQLKPDTFVQHIKRHNIVLKRELGEGAFGKVFLAECYNLCPEQDKILVAVKTLKDASDNARKDFHREAELLTNLQHEHIVKFYGVCVEGDPLIMVFEYMKHGDLNKFLRAHGPDAVLMAEGNPPTELTQSQMLHIAQQIAAGMVYLASQHFVHRDLATRNCLVGENLLVKIGDFGMSRDVYSTDYYRVGGHTMLPIRWMPPESIMYRKFTTESDVWSLGVVLWEIFTYGKQPWYQLSNNEVIECITQGRVLQRPRTCPQEVYELMLGCWQREPHTRKNIKSIHTLLQNLAKASPVYLDILG

SEQ ID NO: 5 - protein, 822 aa, Artificial Sequence
  Synthetic
  MISC_FEATURE (1)..(31): Signal Peptide
  MISC_FEATURE (1)..(31): Rat Sequence
  MISC_FEATURE (32)..(430): Extracellular Domain
  MISC_FEATURE (32)..(432): Human Sequence
  MISC_FEATURE (431)..(454): Transmembrane Domain
  MISC_FEATURE (433)..(822): Rat Sequence
  MISC_FEATURE (455)..(822): Cytoplasmic Domain
MSPWPRWHGPAMARLWGLCLLVLGFWRASLACPTSCKCSASRIWCSDPSPGIVAFPRLEPNSVDPENITEIFIANQKRLEIINEDDVEAYVGLRNLTIVDSGLKFVAHKAFLKNSNLQHINFTRNKLTSLSRKHFRHLDLSELILVGNPFTCSCDIMWIKTLQEAKSSPDTQDLYCLNESSKNIPLANLQIPNCGLPSANLAAPNLTVEEGKSITLSCSVAGDPVPNMYWDVGNLVSKHMNETSHTQGSLRITNISSDDSGKQISCVAENLVGEDQDSVNLTVHFAPTITFLESPTSDHHWCIPFTVKGNPKPALQWFYNGAILNESKYICTKIHVTNHTEYHGCLQLDNPTHMNNGDYTLIAKNEYGKDEKQISAHFMGWPGIDDGANPNYPDVIYEDYGTAANDIGDTTNRSNEIPSTDVTDKTGREHLSVYAVVVIASVVGFCLLVMLLLLKLARHSKFGMKGPASVISNDDDSASPLHHISNGSNTPSSSEGGPDAVIIGMTKIPVIENPQYFGITNSQLKPDTFVQHIKRHNIVLKRELGEGAFGKVFLAECYNLCPEQDKILVAVKTLKDASDNARKDFHREAELLTNLQHEHIVKFYGVCVEGDPLIMVFEYMKHGDLNKFLRAHGPDAVLMAEGNPPTELTQSQMLHIAQQIAAGMVYLASQHFVHRDLATRNCLVGENLLVKIGDFGMSRDVYSTDYYRVGGHTMLPIRWMPPESIMYRKFTTESDVWSLGVVLWEIFTYGKQPWYQLSNNEVIECITQGRVLQRPRTCPQEVYELMLGCWQREPHTRKNIKNIHTLLQNLAKASPVYLDILG

SEQ ID NO: 6 - DNA, 8744 bp, Mus musculus
gtctggagggtgctatgctatgcgtgtgtgcgtgtgtgtgcgcgcgcgcgtgtgtgagcgtgtgtgtttttggatttcatactaattttctggagtttctgcccctgctctgcgtcagccctcacgtcacttcgccagcagtagcagaggcggcggcggcggcggccgccggttagagcccagtcgctgcttcagctgctgttgctgcttctgcagcgctctgctccctgcgcttgctacgggaggccggggaagccgcgcggacagtcctcggtggcctgggccggcactgtcctgctaccgcagttgctccccagccctgaggtgcgcaccgatatcgatattcgtgccggtttagcggttctgcgacccaaagagtccagggagatccaccgagtggtgcctggcgtataggactatgcagccgccttgtggctcggagcagcggcccgcgatgtcccagccactgtgaaccatttggtcagcgccaacctgctcagccccagcaccgacaggctcagcctctggtacgctccactccgcgggaggccaccagcaccaagcagcaagagggcgcagggaaggcctcccccctccggcgggggacgcctggctcagcgtagggacacgcactccgactgactggcactggcagctcgggatgtcgccctggctgaagtggcatggacccgccatggcgcggctctggggcttatgcctgctggtcttgggcttctggagggcctctctcgcctgcccgacgtcctgcaaatgcagttccgctaggatttggtgtactgagccttctccaggcatcgtggcattcccgaggttggaacctaacagcgttgacccggagaacatcacggaaattctcattgcaaaccagaaaaggctagaaatcatcaatgaagatgacgttgaagcttacgtggggctgagaaaccttacaattgtggattccggcttaaagtttgtggcttacaaagcgtttctgaaaaacagcaacctgcggcacataaatttcacacgaaacaagctgacgagtttgtccaggagacatttccgccaccttgacttgtctgacctgatcctgacgggtaatccgttcacgtgctcctgcgacatcatgtggctcaagactctccaggagactaaatccagccccgacactcaggatttgtactgcctcaatgagagcagcaagaacatgcccctggcgaacctgcagatacccaattgtggtctgccatctgcacgtctggctgctcctaacctcaccgtggaggaaggaaagtctgtgaccctttcctgcagtgtggggggtgacccactccccaccttgtactgggacgttgggaatttggtttccaagcacatgaatgaaacaagccacacacagggctccttaaggataacgaacatttcatctgatgacagtggaaagcaaatctcttgtgtggcagaaaaccttgtaggagaagatcaagattctgtgaacctcactgtgcattttgcgccaactatcacgtttctcgagtctccaacctcagatcaccactggtgcattccattcactgtgagaggcaaccccaagcctgcgcttcagtggttctacaatggggccatactgaatgagtccaagtacatctgtactaagatccacgtcaccaatcacacggagtaccatggctgcctccagctggataaccccactcatatgaataacggagactacaccctgatggccaagaacgagtatgggaaggatgagagacagatctccgctcacttcatgggccggcctggagtcgactacgagacaaacccaaattaccctgaagtcctctatgaagactggaccacgccaactgacattggggatactacgaacaaaagtaatgaaatcccctccacggatgttgctgaccaaagcaatcgggagcatctctcggtctatgccgtggtggtgattgcatctgtggtgggattctgcctgctggtgatgttgctcctgctcaagttggcgagacattccaagtttggcatgaaaggcccagcttcggtcatcagcaacgacgatgactctgccagccccctccaccacatctccaatgggagtaacactccatcttcttcggagggcggtcccgacgctgtcattattggaatgaccaagattcctgttattgaaaacccccagtactttggcatcaccaacagtcagctcaagccagacacatttgttcagcatatcaagagacacaacatcgttctgaagagggaacttggggaaggagccttcgggaaagttttccttgccgagtgctacaacctctgcccagagcaggataagatcctggtggctgtgaagacgctgaaggacgccagcgacaatgcacgcaaggactttcatcgggaagctgagctgctgaccaacctccagcacgagcacattgtcaagttctacggtgtctgtgtggagggcgacccactcatcatggtctttgagtacatgaagcacggggacctcaacaagttccttagggcacacgggcccgacgcagtgctgatggcagagggtaacccgcccacagagctgacgcagtcgcagatgctgcacatcgctcagcaaatcgcagcaggtatggtctacctggcgtcccaacactttgtgcaccgtgacctggccacccggaactgcctggtgggagagaacctgctggtgaaaattggggactttgggatgtcccgagatgtgtacagcaccgactactatcgggtcggtggccacacaatgttgcccatccgatggatgcctccagagagcatcatgtacaggaaattcaccaccgagagcgacgtctggagcctgggcgttgtgttgtgggagatcttcacctacggcaagcagccctggtatcagctatcgaacaatgaggtgatagagtgcatcacccagggaagagtccttcagcggcctcgaacgtgtccccaggaggtgtatgagctcatgcttggatgctggcagcgggaaccacacacccggaagaacatcaagagcatccacaccctccttcagaacttggccaaggcatctcccgtctacctggatatcctaggctagggtcctccttctgcccagaccgtccttcccaaggccctcctcagactggcctacacgacgaacctcttgactgccgctgacgtcatgaccttgctgtccttcgctctgacagtgttgacaggaccaggagcggctctttgggggaggcagtgtgtgcttctccatccacagacagtattaactcgcttctggcattgtctctttctctcccttgggtttgtttctttcttttgccccttccccttttatcattatttattcatttatttattttctggtcttcaccgcttcacggccctcagtctctccttgaccaatctggcttctgcattcctattaactgtacatagacaaaggccttaacaaacctaatttgttatatcagcagacactccagtttgcccaccacaactaacaatgccttgttgtattcctgcctttgacgtggatgaaaaaaagggaaaaaaaaatcaaacatctgacttaagctgtcacttccgatgtacagacgtggggcgtttctatggattcacttctatttattatttattaatttatttatttatcactcttcttattgttttctggtggttttaacctatgtgtgagaaggaaaagttgtgtacaatctgggaaaactttatcagtgggaaatgaaaacgagagcgagcaagcgagcaagagagggagagagagagagaagcgttaccataaaccacggcatgagcgagacagagacaagccatgggatcagtcgggagtccgttgtgcttaggaaaacccagcagccattagctgggggagcatgttcggctctgtcccccaagcacctttctgaggaggacacaggatgttgaactctgcttcacgggcagagcttctaatgacagatactggcttgcactggaaagacagttcccacgggacctggacggacaacacatcctacattcagacattgtggtcgggcacggtgacagagttgatccgtttctcaagtgttatctaccaagcttttgtgaagttccatcgaaggaggtagattcttgctcagatataatttcaggaaaacccgagtccttgacaaagacaggagacgctctcaatttggaggcaagtttctcttaccttgaactttttcagacagcaactccgcccagcccccatcttccactctcacctgtcttgtaactgtgcaaacaaaagtgtgcatggtctttgtcaattgatacctatgtgcacgtgtgcagaaactgttgttccagctggggtgtctgattaggagggcagatccataaaaggtctaacctaggcaacttcgggaaaggagaccagatcagtagctggaggcactctccagtaggcggtgaggggtttactgagtaggcatgctgaagcccggatattcacccatctcaaaccccccgggctgcaggacaggcacaggccatccctgaggagaaggggagcccttttgggataccacctgaggttatgttcagtgtgctctggtcaagtcccttgctcggggctctgtttggggagagtggtttcattccaaggtactcattattagtatgctgttttgttaactatactccattaaaaagttaaaaaaaaaaagaattaagccttgacactgtatggctgacaggaggctgtgcccagactgagcctggagatttgcgcccgcacatggtcattggttttccgaaaagagagggtaaatttatatagaaatttacaggtatttgggtagtcatttagaccgagggagaccagtgtttccatttctctgcgccccctctgtgaggggaagttcgatacacttgacacctttataaacggagccagataggaagggagtgacttaattcaccttagaacatttcatttggtgtttatttctgaaggtgcaagagctctgtgtaggtttcatttgtgcccgagcatttctggagcactgtgttttctagcagaaactccgagagccagttctcacaatgaaactttaaaacctgtgtaaattgacagagagcagaaggcgatccaagaggcccactcaagtgagtggtggcacgaggcacatgcggtggccctttctgttgtgctggcccatgagagatgggagctattttgtcctcttcgtccattaaaacaaacccctccagaatacctatagtaatataatgaaagccatatctctgtgatctataccgtcaggtatagatcattaaaggacccatggtactgtcaggcactgtggaaccgtgaggcagcggaaaggcaagggcacatttgtacatgttcctctagcttccgccagccgtgacctatgaactcacataggccggttgctcctagtctgacgggctgccctgggaggaaaagctgcaagatgctcagcagagagcaaaggagaggatagtcttggaaaaggccaaggttggggatgccatacaggattacaccaaagggctgtactgagaatgtgggagcattccattccaggtttgtattttcctcagcaagaaaaaagagcagatagaagggcagaggaggatagagaggaagagaaaggagagggagaagagagcagagaagagagagagagagagagagagagagaatctttatactttttggcaagtcctcgaaggtctcaaaatgaaagtgtctatgcaagtgcaaatttttacagttatttatactaattattattattgttattaattattattattactagtctgttgtctcaagaatatgtgcagatttcagagcattaaagagtatttggtttcttttaaagtagttgggtgagccaaggacaccttaaaataattgtcactgttcatctgctatcgcctttctcatggtattttaagttttagaaaagaaacattcttgttctaaaacatatccctctccatagatgacaaaaaaaaatggtgttagcaaaccgaaacctcccccgattcctgtctgacatccgatccatttctcaactgcttgatgatttccgagcgctttttgcatatgttgtcaaaatattcatattattttggtgagggaatggagactcagaaactcagaggacaaacataagcttcaccgaagtctgtctgccagatacaaactaacatacaaacaagacagccgggaaggaaatgtgctggtagcgtgtctgtggagcagggtgggggttagaacagaaggagacctgggcagtgcacgcagaagagatgttacatcatgtgcttctgctcctggcttctgctgactcccaactttgcgctcagcctcatttagaaaacgcttcaaacactgctcttcagggttctgtcagaactcacacacacgtgctcacaccagccccgcttgtgacgtttttatgtacttctatataaatatatacataatatatgttataaacacttgatttatacatatacaaatgcacacatgtagtgtgtttgtgtgtttatgtataaacatataggctcatggtaatagaataattataagtagggtgcaatatgaataatttgcttaatatttgctaagtaaccaaaactttccaacgtcatgtggcagttcatatttccactctcagtgtgggtaaggatgggctacaccacactttcagctctgtgcagcccttggatggaagatgtgttgaaaaaaaaatcacatcttccctgaaacaactgactgaaagccatcctctacattgaatctgttctctggctctttgcaaaggagaaatgcagacaaatggtctccttgtgtcccagtcctgggaaggagaagtgggttttctcttcttgcacatttgggccgtgctcacctttcctggctctatgccctttacactgggctcagagatgaagcagtctagacccaagctgcagggctgtagggaggcaaatgtcttcgaggctgatagcaaagcatccaaaaatctatagcaagatgcgcagcttgaagtcactcctcatccacacggcaagcaagagccagggcatgcagtgctgtccatctctaggactgggcagtggggtccccggtcaagggcagtctttccctaagcctctccttttgcaaatggcactgccagcagtacctggcattaagtcacgaaaaatttctaaaatggcagcacagacccgtgtgccctcattgctctgcccccacatgcctcatcattagagggctccagttttcaaacttgactttccatttggccctgtatcgtggttaaaggaaatctcaacagagggatggccaattgacctaaatccccagatgtccaagtttgcagtgaaagccagttcttcccaaatgtataactggaatgtagggactcaggttgtgatacttcatacaggaatctcagatgttattgtaaagaactgggttgggagggattcatcactaagccaacaataatgcaggagggcgtggctgatcgttaagccaatagtagtgcaggagggcgtggctgctgtgagggctggaatccatctctgctgctaaagttcagggttctcaactcttttcagctgttgcagcccttcacttctttcccttcggcgttatttatttgtgtatttatttatttatttatttatttatctatctatctatcaacttttggtccattcatcaccaacataaagcaaaaacaattttttacatatatgtaaatgtgttgcaagtgaaacactgtgaatctcacaaccacctcctagcaactatgctgccatcttgacgtgcgtctcaggagtcgagacgggaaaagacgaggacgtcattttgcagcctacgcattctgggccaggtccgtgttcgttttatttctttagtctgtgagttaagaaaacaatccgagtggagggtgacggatgttcggcaagttcggtgaagcagcacgagctctttgcagctataggttcgagcaagaagaaaaaccatgggagatggagaagggaaatttgatggaggggtggggtggggtgggggctctgtcttacagctcgtgtagcttactgttgcttaaaaatgtatacaacagctggaaatgttttcaacacaaggtatttgaaataaatgtgaatcttaaatatgtactcccttaaggaatgaacatattatggtgaaatattgctcccccgcgtcccctacaaatctgcctagagatgtggatacctacatttgcttaagcatcagaccagtgtttgtatatacccgggccatacacactcatctcgacgtctctctgcggatgtatttccccttcactggtgacctggtatttagaactccgtcttttcagttggtttatttccctttaatgtgatgtctctgtgccgattattaccggttcttacttgtttttgcaatccgttttgaggtccagtgttttactgagactcattgcatcttggctgatttcaaagtgacacccgaatacagtgtttaaaaaaaaagtttgtttgtaaatcatgtgaccagcttctctcaccctgacatggaatgtctcttgtactacagtgtatttaataataaaagaaaaaaatgatgtcttacaataaataacatcttccacaagagg

SEQ ID NO: 7 - DNA, 4750 bp, Rattus norvegicus
tgtgcgtgcgtgcgtgtgtgtgtgtgtgtgtgtgtgtgtgtgtgtgtgtgtgtgtgtgtgtgagcgtgtgtgtttttggatttcatactaattttctggagtttctgcccctgctctgcgtcagccctcacgtcacttcgccagcagtagcagaggcggcggcggccgccggttagagcccagtcgctgcttcagctgctgttgctgcttctgcggcgctctgctccctgcgctggctacgggaggccgggggagccgcgccgacagtcctctgtggccagggccggcactgtcctgctaccgcagttgctccccagccctgaggtgcgcaccgatatcgatatccgtgccggtttagcggttctgcgacccaaagagtccagggagagccaccgagtggcgcctggcgtataggaccatgcagccgccttgtggcttggagcagcggcccgtgatgttccagccactgtgaaccatttggtcagcgccaacctgctcagccccagcaccgacaggctcagcctctggtacgctcctctcggcgggaggccatcagcaccaagcagcaagagggctcagggaaggcctcccccctccggcgggggacgcctggctcagcgtagggacacgcactctgactgactggcactggcagctcgggatgtcgccctggccgaggtggcatggacccgccatggcgcggctctggggcttatgcttgctggtcttgggcttctggagggcttctcttgcctgccccatgtcctgcaaatgcagcaccactaggatttggtgtaccgagccttctcctggcatcgtggcatttccgaggttggaacctaacagcattgacccagagaacatcaccgaaattctcattgcaaaccagaaaaggttagaaatcatcaatgaagatgatgtcgaagcttacgtggggctgaaaaaccttacaattgtggattccggcttaaagtttgtggcttacaaggcgtttctgaagaacggcaacctgcggcacatcaatttcactcgaaacaagctgacgagtttgtccaggagacatttccgccaccttgacttgtctgacctgatcctgacgggtaatccgttcacgtgttcctgtgacatcatgtggctcaagactctccaggagacgaaatccagccccgacactcaggatttgtattgcctcaatgagagcagcaagaatacccctctggcgaacctgcagattcccaattgtggtctgccgtctgcacgtctggccgctcctaacctcacggtggaggaagggaagtctgtgaccatttcctgcagcgtcgggggtgacccgctccccaccttgtactgggacgttgggaatttggtttccaaacacatgaatgaaacaagccacacacagggctccttaaggataacaaacatttcatcggatgacagtgggaaacaaatctcttgtgtggcagaaaacctcgttggagaagatcaagactctgtgaacctcactgtgcattttgcaccaaccatcacatttctcgaatctccaacctcagaccaccactggtgcatcccattcactgtgagaggcaaccccaagccagcacttcagtggttctacaacggagccatactgaatgaatccaagtacatctgtaccaaaatacacgtcaccaatcacacggagtaccacggctgcctccagctggataaccccactcatatgaataatggagactacaccctaatggccaagaatgaatatgggaaggacgagagacagatttctgctcacttcatgggccggcctggagttgactatgagacaaacccaaattaccctgaagtcctctatgaagactggaccacgccaactgacatcggggatactacaaacaaaagtaatgagatcccctccacggatgttgctgaccaaaccaatcgggagcatctctcggtctatgccgtggtggtgattgcctctgtggtaggattctgcctgctggtgatgctgcttctgctcaagttggcgagacattccaagtttggcatgaaaggcccagcttccgtcatcagcaacgacgatgactctgccagccctctccaccacatctccaacgggagcaacactccgtcttcttcggagggcgggcccgatgctgtcatcattgggatgaccaagatccctgtcattgaaaacccccagtacttcggtatcaccaacagccagctcaagccggacacatttgttcagcacatcaagagacacaacatcgttctgaagagggagcttggagaaggagcctttgggaaagttttcctagcggagtgctataacctctgccccgagcaggataagatcctggtggccgtgaagacgctgaaggacgccagcgacaatgctcgcaaggactttcatcgcgaagccgagctgctgaccaacctccagcacgagcacattgtcaagttctacggtgtctgtgtggagggcgacccactcatcatggtctttgagtacatgaagcacggggacctcaacaagttccttagggcacacgggccagatgcagtgctgatggcagagggtaacccgcccaccgagctgacgcagtcgcagatgctgcacatcgctcagcaaatcgcagcaggcatggtctacctggcatcccaacacttcgtgcaccgagacctggccacccggaactgcttggtaggagagaacctgctggtgaaaattggggacttcgggatgtcccgggatgtatacagcaccgactactaccgggttggtggccacacaatgttgcccatccgatggatgcctccagagagcatcatgtacaggaaattcaccaccgagagtgacgtctggagcctgggagttgtgttgtgggagatcttcacctacggcaagcagccctggtatcagctatcaaacaacgaggtgatagaatgcatcacccagggcagagtccttcagcggcctcgcacgtgtccccaggaggtgtacgagctgatgctgggatgctggcagcgggaaccacacacaaggaagaacatcaagaacatccacacactccttcagaacttggcgaaggcgtcgcccgtctacctggacatcctaggctagactccctcttctcccagacggcccttcccaaggcacccctcagacctcttaactgccgctgatgtcaccaccttgctgtccttcgctctgacagtgttaacaagacaaggagcggctctccggggtgaggcagtgcgcacttccccatccacagacagtatcgactcgcttctggctttgtcgctttctctccctttggtttgtttctttcttttgcccattctccatttatttatttatttatttatttatttatttatttatttatctatctatctatctatctatctatctatttatttatttattggtcttcactgcttcatggtcctcggcctctctccttgaccgatctggcttctgtactcctattcactgtacatagacaaaggccttaacaaacctgatttgttatatcagcagacactccagtttgcccaccacaactaacaatgccttgttgtattcctgcctttgatgtggatgaaaaaaagggaaaaaaaaataatcaaacatctgacttaaaccgtcacttccgatgtacagacacggggcgtttctatggattcacttctatctatctatttatttatttatctatttatttatttctcttctttgttgttttccggtggttttagcctgtgtatgagaagggaaagtcatgtacagtctgggaaaactttatctgtgggaaatggaaaccagaaagggaaagaagctttaccataaagcacagcaggagtgagacacagaaaagccattggatcagccagagtccgtcctgcataggaaaacccagcagccatcaggctggaggatcatgttcggcactgacccccgaggacctttctgaggaggacacagaatgttaaactctgcatcatggacacagtttccgatcacagatactggccttcaatggaaaaaaaaaaaaacccagatagttcttgtgagacctggacagcacgtccaacatccagacattgtggtcgggcacagtgacagagttgatgcatttctcacgggttattctacagagcttttgtcaagtccaatggaaggaggtagattcttgttcagatatgatttcgggaaaaaccgagtccttgacaaagacaggagacaccctcagttgggaggcaagtttctcttaccttggactttctcacacagcaattctcacccccaccccctccactctcacctgtcttgtaactgtgcaaacaaaagtgtgcatggtctttgtcagttgatacctttgtgcacctctgtgcagaaactgctgtctgtcccggctgtggtacccgatcagtggggtagatccacgaaaggtctcattttaggccgctttgggaaggtaaccagatcggtagctggaagcactctccagtaggtggcgaagggtgagtgggtctgctgaagcctgcatatcttcacccacctcaaacccaccgggctgcacaggggacaggcacaggccacccctgagggacagggaagctctcttgggataccacctgagtttacattcagtgtgctcaggtcaagtctctcgctcggggctctgtttcggggagaatggtttcattccaacgcactcattatcaggattctgttttc

SEQ ID NO: 8 - DNA, 4057 bp, Homo sapiens
gggagcaggagcctcgctggctgcttcgctcgcgctctacgcgctcagtccccggcggtagcaggagcctggacccaggcgccggcggcgggcgtgaggcgccggagcccggcctcgaggtgcataccggacccccattcgcatctaacaaggaatctgcgccccagagagtcccggacgccgccggtcggtgcccggcgcgccgggccatgcagcgacggccgccgcggagctccgagcagcggtagcgcccccctgtaaagcggttcgctatgccgggaccactgtgaaccctgccgcctgccggaacactcttcgctccggaccagctcagcctctgataagctggactcggcacgcccgcaacaagcaccgaggagttaagagagccgcaagcgcagggaaggcctccccgcacgggtgggggaaagcggccggtgcagcgcggggacaggcactcgggctggcactggctgctagggatgtcgtcctggataaggtggcatggacccgccatggcgcggctctggggcttctgctggctggttgtgggcttctggagggccgctttcgcctgtcccacgtcctgcaaatgcagtgcctctcggatctggtgcagcgacccttctcctggcatcgtggcatttccgagattggagcctaacagtgtagatcctgagaacatcaccgaaattttcatcgcaaaccagaaaaggttagaaatcatcaacgaagatgatgttgaagcttatgtgggactgagaaatctgacaattgtggattctggattaaaatttgtggctcataaagcatttctgaaaaacagcaacctgcagcacatcaattttacccgaaacaaactgacgagtttgtctaggaaacatttccgtcaccttgacttgtctgaactgatcctggtgggcaatccatttacatgctcctgtgacattatgtggatcaagactctccaagaggctaaatccagtccagacactcaggatttgtactgcctgaatgaaagcagcaagaatattcccctggcaaacctgcagatacccaattgtggtttgccatctgcaaatctggccgcacctaacctcactgtggaggaaggaaagtctatcacattatcctgtagtgtggcaggtgatccggttcctaatatgtattgggatgttggtaacctggtttccaaacatatgaatgaaacaagccacacacagggctccttaaggataactaacatttcatccgatgacagtgggaagcagatctcttgtgtggcggaaaatcttgtaggagaagatcaagattctgtcaacctcactgtgcattttgcaccaactatcacatttctcgaatctccaacctcagaccaccactggtgcattccattcactgtgaaaggcaaccccaaaccagcgcttcagtggttctataacggggcaatattgaatgagtccaaatacatctgtactaaaatacatgttaccaatcacacggagtaccacggctgcctccagctggataatcccactcacatgaacaatggggactacactctaatagccaagaatgagtatgggaaggatgagaaacagatttctgctcacttcatgggctggcctggaattgacgatggtgcaaacccaaattatcctgatgtaatttatgaagattatggaactgcagcgaatgacatcggggacaccacgaacagaagtaatgaaatcccttccacagacgtcactgataaaaccggtcgggaacatctctcggtctatgctgtggtggtgattgcgtctgtggtgggattttgccttttggtaatgctgtttctgcttaagttggcaagacactccaagtttggcatgaaagatttctcatggtttggatttgggaaagtaaaatcaagacaaggtgttggcccagcctccgttatcagcaatgatgatgactctgccagcccactccatcacatctccaatgggagtaacactccatcttcttcggaaggtggcccagatgctgtcattattggaatgaccaagatccctgtcattgaaaatccccagtactttggcatcaccaacagtcagctcaagccagacacatttgttcagcacatcaagcgacataacattgttctgaaaagggagctaggcgaaggagcctttggaaaagtgttcctagctgaatgctataacctctgtcctgagcaggacaagatcttggtggcagtgaagaccctgaaggatgccagtgacaatgcacgcaaggacttccaccgtgaggccgagctcctgaccaacctccagcatgagcacatcgtcaagttctatggcgtctgcgtggagggcgaccccctcatcatggtctttgagtacatgaagcatggggacctcaacaagttcctcagggcacacggccctgatgccgtgctgatggctgagggcaacccgcccacggaactgacgcagtcgcagatgctgcatatagcccagcagatcgccgcgggcatggtctacctggcgtcccagcacttcgtgcaccgcgatttggccaccaggaactgcctggtcggggagaacttgctggtgaaaatcggggactttgggatgtcccgggacgtgtacagcactgactactacagggtcggtggccacacaatgctgcccattcgctggatgcctccagagagcatcatgtacaggaaattcacgacggaaagcgacgtctggagcctgggggtcgtgttgtgggagattttcacctatggcaaacagccctggtaccagctgtcaaacaatgaggtgatagagtgtatcactcagggccgagtcctgcagcgaccccgcacgtgcccccaggaggtgtatgagctgatgctggggtgctggcagcgagagccccacatgaggaagaacatcaagggcatccataccctccttcagaacttggccaaggcatctccggtctacctggacattctaggctagggcccttttccccagaccgatccttcccaacgtactcctcagacgggctgagaggatgaacatcttttaactgccgctggaggccaccaagctgctctccttcactctgacagtattaacatcaaagactccgagaagctctcgagggaagcagtgtgtacttcttcatccatagacacagtattgacttctttttggcattatctctttctctctttccatctcccttggttgttcctttttctttttttaaattttctttttcttcttttttttcgtcttccctgcttcacgattcttaccctttcttttgaatcaatctggcttctgcattactattaactctgcatagacaaaggccttaacaaacgtaatttgttatatcagcagacactccagtttgcccaccacaactaacaatgccttgttgtattcctgcctttgatgtggatgaaaaaaagggaaaacaaatatttcacttaaactttgtcacttctgctgtacagatatcgagagtttctatggattcacttctatttatttattattattactgttcttattgtttttggatggcttaagcctgtgtataaaaaagaaaacttgtgttcaatctgtgaagcctttatctatgggagattaaaaccagagagaaagaagatttattatgaaccgcaatatgggaggaacaaagacaaccactgggatcagctggtgtcagtccctacttaggaaatactcagcaactgttagctgggaagaatgtattcggcaccttcccctgaggacctttctgaggagtaaaaagactactggcctctgtgccatggatgattcttttcccatcaccagaaatgatagcgtgcagtagagagcaaagatggcttccgtgagacacaagatggcgcatagtgtgctcggacacagttttgtcttcgtaggttgtgatgatagcactggtttgtttctcaagcgctatccacagaacctttgtcaacttcagttgaaaagaggtggattcatgtccagagctcatttcggggtcaggtgggaaagcc

SEQ ID NO: 9 - DNA, 2466 bp, Mus musculus
  misc_feature (1)..(93): Signal Peptide
  misc_feature (94)..(1287): Extracellular Domain
  misc_feature (1288)..(1359): Transmembrane Domain
  misc_feature (1360)..(2463): Cytoplasmic Domain
atgtcgccctggctgaagtggcatggacccgccatggcgcggctctggggcttatgcctgctggtcttgggcttctggagggcctctctcgcctgcccgacgtcctgcaaatgcagttccgctaggatttggtgtactgagccttctccaggcatcgtggcattcccgaggttggaacctaacagcgttgacccggagaacatcacggaaattctcattgcaaaccagaaaaggctagaaatcatcaatgaagatgacgttgaagcttacgtggggctgagaaaccttacaattgtggattccggcttaaagtttgtggcttacaaagcgtttctgaaaaacagcaacctgcggcacataaatttcacacgaaacaagctgacgagtttgtccaggagacatttccgccaccttgacttgtctgacctgatcctgacgggtaatccgttcacgtgctcctgcgacatcatgtggctcaagactctccaggagactaaatccagccccgacactcaggatttgtactgcctcaatgagagcagcaagaacatgcccctggcgaacctgcagatacccaattgtggtctgccatctgcacgtctggctgctcctaacctcaccgtggaggaaggaaagtctgtgaccctttcctgcagtgtggggggtgacccactccccaccttgtactgggacgttgggaatttggtttccaagcacatgaatgaaacaagccacacacagggctccttaaggataacgaacatttcatctgatgacagtggaaagcaaatctcttgtgtggcagaaaaccttgtaggagaagatcaagattctgtgaacctcactgtgcattttgcgccaactatcacgtttctcgagtctccaacctcagatcaccactggtgcattccattcactgtgagaggcaaccccaagcctgcgcttcagtggttctacaatggggccatactgaatgagtccaagtacatctgtactaagatccacgtcaccaatcacacggagtaccatggctgcctccagctggataaccccactcatatgaataacggagactacaccctgatggccaagaacgagtatgggaaggatgagagacagatctccgctcacttcatgggccggcctggagtcgactacgagacaaacccaaattaccctgaagtcctctatgaagactggaccacgccaactgacattggggatactacgaacaaaagtaatgaaatcccctccacggatgttgctgaccaaagcaatcgggagcatctctcggtctatgccgtggtggtgattgcatctgtggtgggattctgcctgctggtgatgttgctcctgctcaagttggcgagacattccaagtttggcatgaaaggcccagcttcggtcatcagcaacgacgatgactctgccagccccctccaccacatctccaatgggagtaacactccatcttcttcggagggcggtcccgacgctgtcattattggaatgaccaagattcctgttattgaaaacccccagtactttggcatcaccaacagtcagctcaagccagacacatttgttcagcatatcaagagacacaacatcgttctgaagagggaacttggggaaggagccttcgggaaagttttccttgccgagtgctacaacctctgcccagagcaggataagatcctggtggctgtgaagacgctgaaggacgccagcgacaatgcacgcaaggactttcatcgggaagctgagctgctgaccaacctccagcacgagcacattgtcaagttctacggtgtctgtgtggagggcgacccactcatcatggtctttgagtacatgaagcacggggacctcaacaagttccttagggcacacgggcccgacgcagtgctgatggcagagggtaacccgcccacagagctgacgcagtcgcagatgctgcacatcgctcagcaaatcgcagcaggtatggtctacctggcgtcccaacactttgtgcaccgtgacctggccacccggaactgcctggtgggagagaacctgctggtgaaaattggggactttgggatgtcccgagatgtgtacagcaccgactactatcgggtcggtggccacacaatgttgcccatccgatggatgcctccagagagcatcatgtacaggaaattcaccaccgagagcgacgtctggagcctgggcgttgtgttgtgggagatcttcacctacggcaagcagccctggtatcagctatcgaacaatgaggtgatagagtgcatcacccagggaagagtccttcagcggcctcgaacgtgtccccaggaggtgtatgagctcatgcttggatgctggcagcgggaaccacacacccggaagaacatcaagagcatccacaccctccttcagaacttggccaaggcatctcccgtctacctggatatcctaggctag

SEQ ID NO: 10 - DNA, 2466 bp, Rattus norvegicus
  misc_feature (1)..(93): Signal Peptide
  misc_feature (94)..(1287): Extracellular Domain
  misc_feature (1288)..(1359): Transmembrane Domain
  misc_feature (1360)..(2463): Cytoplasmic Domain
atgtcgccctggccgaggtggcatggacccgccatggcgcggctctggggcttatgcttgctggtcttgggcttctggagggcttctcttgcctgccccatgtcctgcaaatgcagcaccactaggatttggtgtaccgagccttctcctggcatcgtggcatttccgaggttggaacctaacagcattgacccagagaacatcaccgaaattctcattgcaaaccagaaaaggttagaaatcatcaatgaagatgatgtcgaagcttacgtggggctgaaaaaccttacaattgtggattccggcttaaagtttgtggcttacaaggcgtttctgaagaacggcaacctgcggcacatcaatttcactcgaaacaagctgacgagtttgtccaggagacatttccgccaccttgacttgtctgacctgatcctgacgggtaatccgttcacgtgttcctgtgacatcatgtggctcaagactctccaggagacgaaatccagccccgacactcaggatttgtattgcctcaatgagagcagcaagaatacccctctggcgaacctgcagattcccaattgtggtctgccgtctgcacgtctggccgctcctaacctcacggtggaggaagggaagtctgtgaccatttcctgcagcgtcgggggtgacccgctccccaccttgtactgggacgttgggaatttggtttccaaacacatgaatgaaacaagccacacacagggctccttaaggataacaaacatttcatcggatgacagtgggaaacaaatctcttgtgtggcagaaaacctcgttggagaagatcaagactctgtgaacctcactgtgcattttgcaccaaccatcacatttctcgaatctccaacctcagaccaccactggtgcatcccattcactgtgagaggcaaccccaagccagcacttcagtggttctacaacggagccatactgaatgaatccaagtacatctgtaccaaaatacacgtcaccaatcacacggagtaccacggctgcctccagctggataaccccactcatatgaataatggagactacaccctaatggccaagaatgaatatgggaaggacgagagacagatttctgctcacttcatgggccggcctggagttgactatgagacaaacccaaattaccctgaagtcctctatgaagactggaccacgccaactgacatcggggatactacaaacaaaagtaatgagatcccctccacggatgttgctgaccaaaccaatcgggagcatctctcggtctatgccgtggtggtgattgcctctgtggtaggattctgcctgctggtgatgctgcttctgctcaagttggcgagacattccaagtttggcatgaaaggcccagcttccgtcatcagcaacgacgatgactctgccagccctctccaccacatctccaacgggagcaacactccgtcttcttcggagggcgggcccgatgctgtcatcattgggatgaccaagatccctgtcattgaaaacccccagtacttcggtatcaccaacagccagctcaagccggacacatttgttcagcacatcaagagacacaacatcgttctgaagagggagcttggagaaggagcctttgggaaagttttcctagcggagtgctataacctctgccccgagcaggataagatcctggtggccgtgaagacgctgaaggacgccagcgacaatgctcgcaaggactttcatcgcgaagccgagctgctgaccaacctccagcacgagcacattgtcaagttctacggtgtctgtgtggagggcgacccactcatcatggtctttgagtacatgaagcacggggacctcaacaagttccttagggcacacgggccagatgcagtgctgatggcagagggtaacccgcccaccgagctgacgcagtcgcagatgctgcacatcgctcagcaaatcgcagcaggcatggtctacctggcatcccaacacttcgtgcaccgagacctggccacccggaactgcttggtaggagagaacctgctggtgaaaattggggacttcgggatgtcccgggatgtatacagcaccgactactaccgggttggtggccacacaatgttgcccatccgatggatgcctccagagagcatcatgtacaggaaattcaccaccgagagtgacgtctggagcctgggagttgtgttgtgggagatcttcacctacggcaagcagccctggtatcagctatcaaacaacgaggtgatagaatgcatcacccagggcagagtccttcagcggcctcgcacgtgtccccaggaggtgtacgagctgatgctgggatgctggcagcgggaaccacacacaaggaagaacatcaagaacatccacacactccttcagaacttggcgaaggcgtcgcccgtctacctggacatcctaggctag

SEQ ID NO: 11 - DNA, 2517 bp, Homo sapiens
  misc_feature (1)..(93): Signal Peptide
  misc_feature (94)..(1290): Extracellular Domain
  misc_feature (1291)..(1362): Transmembrane Domain
  misc_feature (1363)..(2514): Cytoplasmic Domain
atgtcgtcctggataaggtggcatggacccgccatggcgcggctctggggcttctgctggctggttgtgggcttctggagggccgctttcgcctgtcccacgtcctgcaaatgcagtgcctctcggatctggtgcagcgacccttctcctggcatcgtggcatttccgagattggagcctaacagtgtagatcctgagaacatcaccgaaattttcatcgcaaaccagaaaaggttagaaatcatcaacgaagatgatgttgaagcttatgtgggactgagaaatctgacaattgtggattctggattaaaatttgtggctcataaagcatttctgaaaaacagcaacctgcagcacatcaattttacccgaaacaaactgacgagtttgtctaggaaacatttccgtcaccttgacttgtctgaactgatcctggtgggcaatccatttacatgctcctgtgacattatgtggatcaagactctccaagaggctaaatccagtccagacactcaggatttgtactgcctgaatgaaagcagcaagaatattcccctggcaaacctgcagatacccaattgtggtttgccatctgcaaatctggccgcacctaacctcactgtggaggaaggaaagtctatcacattatcctgtagtgtggcaggtgatccggttcctaatatgtattgggatgttggtaacctggtttccaaacatatgaatgaaacaagccacacacagggctccttaaggataactaacatttcatccgatgacagtgggaagcagatctcttgtgtggcggaaaatcttgtaggagaagatcaagattctgtcaacctcactgtgcattttgcaccaactatcacatttctcgaatctccaacctcagaccaccactggtgcattccattcactgtgaaaggcaaccccaaaccagcgcttcagtggttctataacggggcaatattgaatgagtccaaatacatctgtactaaaatacatgttaccaatcacacggagtaccacggctgcctccagctggataatcccactcacatgaacaatggggactacactctaatagccaagaatgagtatgggaaggatgagaaacagatttctgctcacttcatgggctggcctggaattgacgatggtgcaaacccaaattatcctgatgtaatttatgaagattatggaactgcagcgaatgacatcggggacaccacgaacagaagtaatgaaatcccttccacagacgtcactgataaaaccggtcgggaacatctctcggtctatgctgtggtggtgattgcgtctgtggtgggattttgccttttggtaatgctgtttctgcttaagttggcaagacactccaagtttggcatgaaagatttctcatggtttggatttgggaaagtaaaatcaagacaaggtgttggcccagcctccgttatcagcaatgatgatgactctgccagcccactccatcacatctccaatgggagtaacactccatcttcttcggaaggtggcccagatgctgtcattattggaatgaccaagatccctgtcattgaaaatccccagtactttggcatcaccaacagtcagctcaagccagacacatttgttcagcacatcaagcgacataacattgttctgaaaagggagctaggcgaaggagcctttggaaaagtgttcctagctgaatgctataacctctgtcctgagcaggacaagatcttggtggcagtgaagaccctgaaggatgccagtgacaatgcacgcaaggacttccaccgtgaggccgagctcctgaccaacctccagcatgagcacatcgtcaagttctatggcgtctgcgtggagggcgaccccctcatcatggtctttgagtacatgaagcatggggacctcaacaagttcctcagggcacacggccctgatgccgtgctgatggctgagggcaacccgcccacggaactgacgcagtcgcagatgctgcatatagcccagcagatcgccgcgggcatggtctacctggcgtcccagcacttcgtgcaccgcgatttggccaccaggaactgcctggtcggggagaacttgctggtgaaaatcggggactttgggatgtcccgggacgtgtacagcactgactactacagggtcggtggccacacaatgctgcccattcgctggatgcctccagagagcatcatgtacaggaaattcacgacggaaagcgacgtctggagcctgggggtcgtgttgtgggagattttcacctatggcaaacagccctggtaccagctgtcaaacaatgaggtgatagagtgtatcactcagggccgagtcctgcagcgaccccgcacgtgcccccaggaggtgtatgagctgatgctggggtgctggcagcgagagccccacatgaggaagaacatcaagggcatccataccctccttcagaacttggccaaggcatctccggtctacctggacattctaggctag

SEQ ID NO: 12 - DNA, 2469 bp, Artificial Sequence
  Synthetic
  misc_feature (1)..(93): Signal Peptide
  misc_feature (1)..(93): Mouse Sequence
  misc_feature (94)..(1290): Extracellular Domain
  misc_feature (94)..(1296): Human Sequence
  misc_feature (1291)..(1362): Transmembrane Domain
  misc_feature (1297)..(2466): Mouse Sequence
  misc_feature (1363)..(2466): Cytoplasmic Domain
atgtcgccctggctgaagtggcatggacccgccatggcgcggctctggggcttatgcctgctggtcttgggcttctggagggcctctctcgcctgtcccacgtcctgcaaatgcagtgcctctcggatctggtgcagcgacccttctcctggcatcgtggcatttccgagattggagcctaacagtgtagatcctgagaacatcaccgaaattttcatcgcaaaccagaaaaggttagaaatcatcaacgaagatgatgttgaagcttatgtgggactgagaaatctgacaattgtggattctggattaaaatttgtggctcataaagcatttctgaaaaacagcaacctgcagcacatcaattttacccgaaacaaactgacgagtttgtctaggaaacatttccgtcaccttgacttgtctgaactgatcctggtgggcaatccatttacatgctcctgtgacattatgtggatcaagactctccaagaggctaaatccagtccagacactcaggatttgtactgcctgaatgaaagcagcaagaatattcccctggcaaacctgcagatacccaattgtggtttgccatctgcaaatctggccgcacctaacctcactgtggaggaaggaaagtctatcacattatcctgtagtgtggcaggtgatccggttcctaatatgtattgggatgttggtaacctggtttccaaacatatgaatgaaacaagccacacacagggctccttaaggataactaacatttcatccgatgacagtgggaagcagatctcttgtgtggcggaaaatcttgtaggagaagatcaagattctgtcaacctcactgtgcattttgcaccaactatcacatttctcgaatctccaacctcagaccaccactggtgcattccattcactgtgaaaggcaaccccaaaccagcgcttcagtggttctataacggggcaatattgaatgagtccaaatacatctgtactaaaatacatgttaccaatcacacggagtaccacggctgcctccagctggataatcccactcacatgaacaatggggactacactctaatagccaagaatgagtatgggaaggatgagaaacagatttctgctcacttcatgggctggcctggaattgacgatggtgcaaacccaaattatcctgatgtaatttatgaagattatggaactgcagcgaatgacatcggggacaccacgaacagaagtaatgaaatcccttccacagacgtcactgataaaaccggtcgggaacatctctcggtctatgccgtggtggtgattgcatctgtggtgggattctgcctgctggtgatgttgctcctgctcaagttggcgagacattccaagtttggcatgaaaggcccagcttcggtcatcagcaacgacgatgactctgccagccccctccaccacatctccaatgggagtaacactccatcttcttcggagggcggtcccgacgctgtcattattggaatgaccaagattcctgttattgaaaacccccagtactttggcatcaccaacagtcagctcaagccagacacatttgttcagcatatcaagagacacaacatcgttctgaagagggaacttggggaaggagccttcgggaaagttttccttgccgagtgctacaacctctgcccagagcaggataagatcctggtggctgtgaagacgctgaaggacgccagcgacaatgcacgcaaggactttcatcgggaagctgagctgctgaccaacctccagcacgagcacattgtcaagttctacggtgtctgtgtggagggcgacccactcatcatggtctttgagtacatgaagcacggggacctcaacaagttccttagggcacacgggcccgacgcagtgctgatggcagagggtaacccgcccacagagctgacgcagtcgcagatgctgcacatcgctcagcaaatcgcagcaggtatggtctacctggcgtcccaacactttgtgcaccgtgacctggccacccggaactgcctggtgggagagaacctgctggtgaaaattggggactttgggatgtcccgagatgtgtacagcaccgactactatcgggtcggtggccacacaatgttgcccatccgatggatgcctccagagagcatcatgtacaggaaattcaccaccgagagcgacgtctggagcctgggcgttgtgttgtgggagatcttcacctacggcaagcagccctggtatcagctatcgaacaatgaggtgatagagtgcatcacccagggaagagtccttcagcggcctcgaacgtgtccccaggaggtgtatgagctcatgcttggatgctggcagcgggaaccacacacccggaagaacatcaagagcatccacaccctccttcagaacttggccaaggcatctcccgtctacctggatatcctaggctag

SEQ ID NO: 13 - DNA, 2469 bp, Artificial Sequence
  Synthetic
  misc_feature (1)..(93): Signal Peptide
  misc_feature (1)..(93): Rat Sequence
  misc_feature (94)..(1290): Extracellular Domain
  misc_feature (94)..(1296): Human Sequence
  misc_feature (1291)..(1362): Transmembrane Domain
  misc_feature (1297)..(2466): Rat Sequence
  misc_feature (1363)..(2466): Cytoplasmic Domain
atgtcgccctggccgaggtggcatggacccgccatggcgcggctctggggcttatgcttgctggtcttgggcttctggagggcttctcttgcctgtcccacgtcctgcaaatgcagtgcctctcggatctggtgcagcgacccttctcctggcatcgtggcatttccgagattggagcctaacagtgtagatcctgagaacatcaccgaaattttcatcgcaaaccagaaaaggttagaaatcatcaacgaagatgatgttgaagcttatgtgggactgagaaatctgacaattgtggattctggattaaaatttgtggctcataaagcatttctgaaaaacagcaacctgcagcacatcaattttacccgaaacaaactgacgagtttgtctaggaaacatttccgtcaccttgacttgtctgaactgatcctggtgggcaatccatttacatgctcctgtgacattatgtggatcaagactctccaagaggctaaatccagtccagacactcaggatttgtactgcctgaatgaaagcagcaagaatattcccctggcaaacctgcagatacccaattgtggtttgccatctgcaaatctggccgcacctaacctcactgtggaggaaggaaagtctatcacattatcctgtagtgtggcaggtgatccggttcctaatatgtattgggatgttggtaacctggtttccaaacatatgaatgaaacaagccacacacagggctccttaaggataactaacatttcatccgatgacagtgggaagcagatctcttgtgtggcggaaaatcttgtaggagaagatcaagattctgtcaacctcactgtgcattttgcaccaactatcacatttctcgaatctccaacctcagaccaccactggtgcattccattcactgtgaaaggcaaccccaaaccagcgcttcagtggttctataacggggcaatattgaatgagtccaaatacatctgtactaaaatacatgttaccaatcacacggagtaccacggctgcctccagctggataatcccactcacatgaacaatggggactacactctaatagccaagaatgagtatgggaaggatgagaaacagatttctgctcacttcatgggctggcctggaattgacgatggtgcaaacccaaattatcctgatgtaatttatgaagattatggaactgcagcgaatgacatcggggacaccacgaacagaagtaatgaaatcccttccacagacgtcactgataaaaccggtcgggaacatctctcggtctatgccgtggtggtgattgcctctgtggtaggattctgcctgctggtgatgctgcttctgctcaagttggcgagacattccaagtttggcatgaaaggcccagcttccgtcatcagcaacgacgatgactctgccagccctctccaccacatctccaacgggagcaacactccgtcttcttcggagggcgggcccgatgctgtcatcattgggatgaccaagatccctgtcattgaaaacccccagtacttcggtatcaccaacagccagctcaagccggacacatttgttcagcacatcaagagacacaacatcgttctgaagagggagcttggagaaggagcctttgggaaagttttcctagcggagtgctataacctctgccccgagcaggataagatcctggtggccgtgaagacgctgaaggacgccagcgacaatgctcgcaaggactttcatcgcgaagccgagctgctgaccaacctccagcacgagcacattgtcaagttctacggtgtctgtgtggagggcgacccactcatcatggtctttgagtacatgaagcacggggacctcaacaagttccttagggcacacgggccagatgcagtgctgatggcagagggtaacccgcccaccgagctgacgcagtcgcagatgctgcacatcgctcagcaaatcgcagcaggcatggtctacctggcatcccaacacttcgtgcaccgagacctggccacccggaactgcttggtaggagagaacctgctggtgaaaattggggacttcgggatgtcccgggatgtatacagcaccgactactaccgggttggtggccacacaatgttgcccatccgatggatgcctccagagagcatcatgtacaggaaattcaccaccgagagtgacgtctggagcctgggagttgtgttgtgggagatcttcacctacggcaagcagccctggtatcagctatcaaacaacgaggtgatagaatgcatcacccagggcagagtccttcagcggcctcgcacgtgtccccaggaggtgtacgagctgatgctgggatgctggcagcgggaaccacacacaaggaagaacatcaagaacatccacacactccttcagaacttggcgaaggcgtcgcccgtctacctggacatcctaggctag

SEQ ID NO: 14 - DNA, 22 bp, Artificial Sequence
  Synthetic
aggtgggtaggtcctggaagtg

SEQ ID NO: 15 - DNA, 20 bp, Artificial Sequence
  Synthetic
aatgctgtcccaagagtggg

SEQ ID NO: 16 - DNA, 21 bp, Artificial Sequence
  Synthetic
gtcctgcatcccttgtctttg

SEQ ID NO: 17 - DNA, 21 bp, Artificial Sequence
  Synthetic
atgtgggcgttgtgcagtctc

SEQ ID NO: 18 - DNA, 24 bp, Artificial Sequence
  Synthetic
cgctgcagtgcattgaactcagca

SEQ ID NO: 19 - DNA, 20 bp, Artificial Sequence
  Synthetic
ctgtggagggacgtgaccag

SEQ ID NO: 20 - DNA, 22 bp, Artificial Sequence
  Synthetic
tccgctaggatttggtgtactg

SEQ ID NO: 21 - DNA, 24 bp, Artificial Sequence
  Synthetic
agccttctccaggcatcgtggcat

SEQ ID NO: 22 - DNA, 19 bp, Artificial Sequence
  Synthetic
tccgggtcaacgctgttag

SEQ ID NO: 23 - DNA, 18 bp, Artificial Sequence
  Synthetic
tcctgcgagggttctgac

SEQ ID NO: 24 - DNA, 29 bp, Artificial Sequence
  Synthetic
tgggtgctcatatgccagagaaattgtca

SEQ ID NO: 25 - DNA, 22 bp, Artificial Sequence
  Synthetic
cgatctgtgatggcctgcttac

SEQ ID NO: 26 - DNA, 22 bp, Artificial Sequence
  Synthetic
gggctcaggcaggtatatgttg

SEQ ID NO: 27 - DNA, 27 bp, Artificial Sequence
  Synthetic
acagatgctgtcccaaacatagcaaga

SEQ ID NO: 28 - DNA, 23 bp, Artificial Sequence
  Synthetic
ccaaccctaagccagtgaaacag

SEQ ID NO: 29 - DNA, 20 bp, Artificial Sequence
  Synthetic
gtgctggagaccaggagact

SEQ ID NO: 30 - DNA, 28 bp, Artificial Sequence
  Synthetic
tgccatactcagtttatacggtgctgac

SEQ ID NO: 31 - DNA, 20 bp, Artificial Sequence
  Synthetic
gcctggtggctcagtcaatg

SEQ ID NO: 32 - DNA, 19 bp, Artificial Sequence
  Synthetic
gcagacactggatgggtca

SEQ ID NO: 33 - DNA, 26 bp, Artificial Sequence
  Synthetic
ccattcgcgagttatgagaagctgca

SEQ ID NO: 34 - DNA, 22 bp, Artificial Sequence
  Synthetic
acagggttagctggtgaatgga

SEQ ID NO: 35 - DNA, 19 bp, Artificial Sequence
  Synthetic
tcggagcacaggactacag

SEQ ID NO: 36 - DNA, 25 bp, Artificial Sequence
  Synthetic
caagaggaactgtgtccaggaaagc

SEQ ID NO: 37 - DNA, 22 bp, Artificial Sequence
  Synthetic
agcgtgcctcacctaacctcta

SEQ ID NO: 38 - DNA, 19 bp, Artificial Sequence
  Synthetic
gcacagcactgtaaaggca

SEQ ID NO: 39 - DNA, 29 bp, Artificial Sequence
  Synthetic
acggaactcgaaggaattggtattgttgt

SEQ ID NO: 40 - DNA, 23 bp, Artificial Sequence
  Synthetic
acacagctatgggagaaagactg

SEQ ID NO: 41 - DNA, 23 bp, Artificial Sequence
  Synthetic
ccggttggcgagtgcgcatgcac

SEQ ID NO: 42 - DNA, 23 bp, Artificial Sequence
  Synthetic
ccttccggttggcgagtgcgcat

SEQ ID NO: 43 - DNA, 23 bp, Artificial Sequence
  Synthetic
ccaagggtgcgttgatggatcta

SEQ ID NO: 44 - DNA, 23 bp, Artificial Sequence
  Synthetic
gaatgccaagggtgcgttgatgg

SEQ ID NO: 45 - DNA, 23 bp, Artificial Sequence
  Synthetic
ctgggtgattgggactgagaaag

SEQ ID NO: 46 - DNA, 24 bp, Artificial Sequence
  Synthetic
cagccttgaaagtatggcttgggc

SEQ ID NO: 47 - DNA, 18 bp, Artificial Sequence
  Synthetic
gcactcgccaaccggaag

SEQ ID NO: 48 - DNA, 23 bp, Artificial Sequence
  Synthetic
gaccagctcacccttacttatgg

SEQ ID NO: 49 - DNA, 23 bp, Artificial Sequence
  Synthetic
actgaatgccaagggtgcgttga

SEQ ID NO: 50 - DNA, 23 bp, Artificial Sequence
  Synthetic
tcttggaaatccgctgaagagtt

SEQ ID NO: 51 - protein, 31 aa, Mus musculus
MSPWLKWHGPAMARLWGLCLLVLGFWRASLA

SEQ ID NO: 52 - protein, 398 aa, Mus musculus
CPTSCKCSSARIWCTEPSPGIVAFPRLEPNSVDPENITEILIANQKRLEIINEDDVEAYVGLRNLTIVDSGLKFVAYKAFLKNSNLRHINFTRNKLTSLSRRHFRHLDLSDLILTGNPFTCSCDIMWLKTLQETKSSPDTQDLYCLNESSKNMPLANLQIPNCGLPSARLAAPNLTVEEGKSVTLSCSVGGDPLPTLYWDVGNLVSKHMNETSHTQGSLRITNISSDDSGKQISCVAENLVGEDQDSVNLTVHFAPTITFLESPTSDHHWCIPFTVRGNPKPALQWFYNGAILNESKYICTKIHVTNHTEYHGCLQLDNPTHMNNGDYTLMAKNEYGKDERQISAHFMGRPGVDYETNPNYPEVLYEDWTTPTDIGDTTNKSNEIPSTDVADQSNREH

SEQ ID NO: 53 - protein, 24 aa, Mus musculus
LSVYAVVVIASVVGFCLLVMLLLL

SEQ ID NO: 54 - protein, 368 aa, Mus musculus
KLARHSKFGMKGPASVISNDDDSASPLHHISNGSNTPSSSEGGPDAVIIGMTKIPVIENPQYFGITNSQLKPDTFVQHIKRHNIVLKRELGEGAFGKVFLAECYNLCPEQDKILVAVKTLKDASDNARKDFHREAELLTNLQHEHIVKFYGVCVEGDPLIMVFEYMKHGDLNKFLRAHGPDAVLMAEGNPPTELTQSQMLHIAQQIAAGMVYLASQHFVHRDLATRNCLVGENLLVKIGDFGMSRDVYSTDYYRVGGHTMLPIRWMPPESIMYRKFTTESDVWSLGVVLWEIFTYGKQPWYQLSNNEVIECITQGRVLQRPRTCPQEVYELMLGCWQREPHTRKNIKSIHTLLQNLAKASPVYLDILG

SEQ ID NO: 55 - protein, 31 aa, Rattus norvegicus
MSPWPRWHGPAMARLWGLCLLVLGFWRASLA

SEQ ID NO: 56 - protein, 398 aa, Rattus norvegicus
CPMSCKCSTTRIWCTEPSPGIVAFPRLEPNSIDPENITEILIANQKRLEIINEDDVEAYVGLKNLTIVDSGLKFVAYKAFLKNGNLRHINFTRNKLTSLSRRHFRHLDLSDLILTGNPFTCSCDIMWLKTLQETKSSPDTQDLYCLNESSKNTPLANLQIPNCGLPSARLAAPNLTVEEGKSVTISCSVGGDPLPTLYWDVGNLVSKHMNETSHTQGSLRITNISSDDSGKQISCVAENLVGEDQDSVNLTVHFAPTITFLESPTSDHHWCIPFTVRGNPKPALQWFYNGAILNESKYICTKIHVTNHTEYHGCLQLDNPTHMNNGDYTLMAKNEYGKDERQISAHFMGRPGVDYETNPNYPEVLYEDWTTPTDIGDTTNKSNEIPSTDVADQTNREH

SEQ ID NO: 57 - protein, 24 aa, Rattus norvegicus
LSVYAVVVIASVVGFCLLVMLLLL

SEQ ID NO: 58 - protein, 368 aa, Rattus norvegicus
KLARHSKFGMKGPASVISNDDDSASPLHHISNGSNTPSSSEGGPDAVIIGMTKIPVIENPQYFGITNSQLKPDTFVQHIKRHNIVLKRELGEGAFGKVFLAECYNLCPEQDKILVAVKTLKDASDNARKDFHREAELLTNLQHEHIVKFYGVCVEGDPLIMVFEYMKHGDLNKFLRAHGPDAVLMAEGNPPTELTQSQMLHIAQQIAAGMVYLASQHFVHRDLATRNCLVGENLLVKIGDFGMSRDVYSTDYYRVGGHTMLPIRWMPPESIMYRKFTTESDVWSLGVVLWEIFTYGKQPWYQLSNNEVIECITQGRVLQRPRTCPQEVYELMLGCWQREPHTRKNIKNIHTLLQNLAKASPVYLDILG

SEQ ID NO: 59 - protein, 31 aa, Homo sapiens
MSSWIRWHGPAMARLWGFCWLVVGFWRAAFA

SEQ ID NO: 60 - protein, 399 aa, Homo sapiens
CPTSCKCSASRIWCSDPSPGIVAFPRLEPNSVDPENITEIFIANQKRLEIINEDDVEAYVGLRNLTIVDSGLKFVAHKAFLKNSNLQHINFTRNKLTSLSRKHFRHLDLSELILVGNPFTCSCDIMWIKTLQEAKSSPDTQDLYCLNESSKNIPLANLQIPNCGLPSANLAAPNLTVEEGKSITLSCSVAGDPVPNMYWDVGNLVSKHMNETSHTQGSLRITNISSDDSGKQISCVAENLVGEDQDSVNLTVHFAPTITFLESPTSDHHWCIPFTVKGNPKPALQWFYNGAILNESKYICTKIHVTNHTEYHGCLQLDNPTHMNNGDYTLIAKNEYGKDEKQISAHFMGWPGIDDGANPNYPDVIYEDYGTAANDIGDTTNRSNEIPSTDVTDKTGREH

SEQ ID NO: 61 - protein, 24 aa, Homo sapiens
LSVYAVVVIASVVGFCLLVMLFLL

SEQ ID NO: 62 - protein, 384 aa, Homo sapiens
KLARHSKFGMKDFSWFGFGKVKSRQGVGPASVISNDDDSASPLHHISNGSNTPSSSEGGPDAVIIGMTKIPVIENPQYFGITNSQLKPDTFVQHIKRHNIVLKRELGEGAFGKVFLAECYNLCPEQDKILVAVKTLKDASDNARKDFHREAELLTNLQHEHIVKFYGVCVEGDPLIMVFEYMKHGDLNKFLRAHGPDAVLMAEGNPPTELTQSQMLHIAQQIAAGMVYLASQHFVHRDLATRNCLVGENLLVKIGDFGMSRDVYSTDYYRVGGHTMLPIRWMPPESIMYRKFTTESDVWSLGVVLWEIFTYGKQPWYQLSNNEVIECITQGRVLQRPRTCPQEVYELMLGCWQREPHMRKNIKGIHTLLQNLAKASPVYLDILG

SEQ ID NO: 63 - DNA, 93 bp, Mus musculus
atgtcgccctggctgaagtggcatggacccgccatggcgcggctctggggcttatgcctgctggtcttgggcttctggagggcctctctcgcc

SEQ ID NO: 64 - DNA, 1194 bp, Mus musculus
tgcccgacgtcctgcaaatgcagttccgctaggatttggtgtactgagccttctccaggcatcgtggcattcccgaggttggaacctaacagcgttgacccggagaacatcacggaaattctcattgcaaaccagaaaaggctagaaatcatcaatgaagatgacgttgaagcttacgtggggctgagaaaccttacaattgtggattccggcttaaagtttgtggcttacaaagcgtttctgaaaaacagcaacctgcggcacataaatttcacacgaaacaagctgacgagtttgtccaggagacatttccgccaccttgacttgtctgacctgatcctgacgggtaatccgttcacgtgctcctgcgacatcatgtggctcaagactctccaggagactaaatccagccccgacactcaggatttgtactgcctcaatgagagcagcaagaacatgcccctggcgaacctgcagatacccaattgtggtctgccatctgcacgtctggctgctcctaacctcaccgtggaggaaggaaagtctgtgaccctttcctgcagtgtggggggtgacccactccccaccttgtactgggacgttgggaatttggtttccaagcacatgaatgaaacaagccacacacagggctccttaaggataacgaacatttcatctgatgacagtggaaagcaaatctcttgtgtggcagaaaaccttgtaggagaagatcaagattctgtgaacctcactgtgcattttgcgccaactatcacgtttctcgagtctccaacctcagatcaccactggtgcattccattcactgtgagaggcaaccccaagcctgcgcttcagtggttctacaatggggccatactgaatgagtccaagtacatctgtactaagatccacgtcaccaatcacacggagtaccatggctgcctccagctggataaccccactcatatgaataacggagactacaccctgatggccaagaacgagtatgggaaggatgagagacagatctccgctcacttcatgggccggcctggagtcgactacgagacaaacccaaattaccctgaagtcctctatgaagactggaccacgccaactgacattggggatactacgaacaaaagtaatgaaatcccctccacggatgttgctgaccaaagcaatcgggagcat

SEQ ID NO: 65 - DNA, 72 bp, Mus musculus
ctctcggtctatgccgtggtggtgattgcatctgtggtgggattctgcctgctggtgatgttgctcctgctc

SEQ ID NO: 66 - DNA, 1104 bp, Mus musculus
aagttggcgagacattccaagtttggcatgaaaggcccagcttcggtcatcagcaacgacgatgactctgccagccccctccaccacatctccaatgggagtaacactccatcttcttcggagggcggtcccgacgctgtcattattggaatgaccaagattcctgttattgaaaacccccagtactttggcatcaccaacagtcagctcaagccagacacatttgttcagcatatcaagagacacaacatcgttctgaagagggaacttggggaaggagccttcgggaaagttttccttgccgagtgctacaacctctgcccagagcaggataagatcctggtggctgtgaagacgctgaaggacgccagcgacaatgcacgcaaggactttcatcgggaagctgagctgctgaccaacctccagcacgagcacattgtcaagttctacggtgtctgtgtggagggcgacccactcatcatggtctttgagtacatgaagcacggggacctcaacaagttccttagggcacacgggcccgacgcagtgctgatggcagagggtaacccgcccacagagctgacgcagtcgcagatgctgcacatcgctcagcaaatcgcagcaggtatggtctacctggcgtcccaacactttgtgcaccgtgacctggccacccggaactgcctggtgggagagaacctgctggtgaaaattggggactttgggatgtcccgagatgtgtacagcaccgactactatcgggtcggtggccacacaatgttgcccatccgatggatgcctccagagagcatcatgtacaggaaattcaccaccgagagcgacgtctggagcctgggcgttgtgttgtgggagatcttcacctacggcaagcagccctggtatcagctatcgaacaatgaggtgatagagtgcatcacccagggaagagtccttcagcggcctcgaacgtgtccccaggaggtgtatgagctcatgcttggatgctggcagcgggaaccacacacccggaagaacatcaagagcatccacaccctccttcagaacttggccaaggcatctcccgtctacctggatatcctaggc

SEQ ID NO: 67 - DNA, 93 bp, Rattus norvegicus
atgtcgccctggccgaggtggcatggacccgccatggcgcggctctggggcttatgcttgctggtcttgggcttctggagggcttctcttgcc

SEQ ID NO: 68 - DNA, 1194 bp, Rattus norvegicus
tgccccatgtcctgcaaatgcagcaccactaggatttggtgtaccgagccttctcctggcatcgtggcatttccgaggttggaacctaacagcattgacccagagaacatcaccgaaattctcattgcaaaccagaaaaggttagaaatcatcaatgaagatgatgtcgaagcttacgtggggctgaaaaaccttacaattgtggattccggcttaaagtttgtggcttacaaggcgtttctgaagaacggcaacctgcggcacatcaatttcactcgaaacaagctgacgagtttgtccaggagacatttccgccaccttgacttgtctgacctgatcctgacgggtaatccgttcacgtgttcctgtgacatcatgtggctcaagactctccaggagacgaaatccagccccgacactcaggatttgtattgcctcaatgagagcagcaagaatacccctctggcgaacctgcagattcccaattgtggtctgccgtctgcacgtctggccgctcctaacctcacggtggaggaagggaagtctgtgaccatttcctgcagcgtcgggggtgacccgctccccaccttgtactgggacgttgggaatttggtttccaaacacatgaatgaaacaagccacacacagggctccttaaggataacaaacatttcatcggatgacagtgggaaacaaatctcttgtgtggcagaaaacctcgttggagaagatcaagactctgtgaacctcactgtgcattttgcaccaaccatcacatttctcgaatctccaacctcagaccaccactggtgcatcccattcactgtgagaggcaaccccaagccagcacttcagtggttctacaacggagccatactgaatgaatccaagtacatctgtaccaaaatacacgtcaccaatcacacggagtaccacggctgcctccagctggataaccccactcatatgaataatggagactacaccctaatggccaagaatgaatatgggaaggacgagagacagatttctgctcacttcatgggccggcctggagttgactatgagacaaacccaaattaccctgaagtcctctatgaagactggaccacgccaactgacatcggggatactacaaacaaaagtaatgagatcccctccacggatgttgctgaccaaaccaatcgggagcat

SEQ ID NO: 69 - DNA, 72 bp, Rattus norvegicus
ctctcggtctatgccgtggtggtgattgcctctgtggtaggattctgcctgctggtgatgctgcttctgctc

SEQ ID NO: 70 - DNA, 1104 bp, Rattus norvegicus
aagttggcgagacattccaagtttggcatgaaaggcccagcttccgtcatcagcaacgacgatgactctgccagccctctccaccacatctccaacgggagcaacactccgtcttcttcggagggcgggcccgatgctgtcatcattgggatgaccaagatccctgtcattgaaaacccccagtacttcggtatcaccaacagccagctcaagccggacacatttgttcagcacatcaagagacacaacatcgttctgaagagggagcttggagaaggagcctttgggaaagttttcctagcggagtgctataacctctgccccgagcaggataagatcctggtggccgtgaagacgctgaaggacgccagcgacaatgctcgcaaggactttcatcgcgaagccgagctgctgaccaacctccagcacgagcacattgtcaagttctacggtgtctgtgtggagggcgacccactcatcatggtctttgagtacatgaagcacggggacctcaacaagttccttagggcacacgggccagatgcagtgctgatggcagagggtaacccgcccaccgagctgacgcagtcgcagatgctgcacatcgctcagcaaatcgcagcaggcatggtctacctggcatcccaacacttcgtgcaccgagacctggccacccggaactgcttggtaggagagaacctgctggtgaaaattggggacttcgggatgtcccgggatgtatacagcaccgactactaccgggttggtggccacacaatgttgcccatccgatggatgcctccagagagcatcatgtacaggaaattcaccaccgagagtgacgtctggagcctgggagttgtgttgtgggagatcttcacctacggcaagcagccctggtatcagctatcaaacaacgaggtgatagaatgcatcacccagggcagagtccttcagcggcctcgcacgtgtccccaggaggtgtacgagctgatgctgggatgctggcagcgggaaccacacacaaggaagaacatcaagaacatccacacactccttcagaacttggcgaaggcgtcgcccgtctacctggacatcctaggc

SEQ ID NO: 71 - DNA, 93 bp, Homo sapiens
atgtcgtcctggataaggtggcatggacccgccatggcgcggctctggggcttctgctggctggttgtgggcttctggagggccgctttcgcc

SEQ ID NO: 72 - DNA, 1197 bp, Homo sapiens
tgtcccacgtcctgcaaatgcagtgcctctcggatctggtgcagcgacccttctcctggcatcgtggcatttccgagattggagcctaacagtgtagatcctgagaacatcaccgaaattttcatcgcaaaccagaaaaggttagaaatcatcaacgaagatgatgttgaagcttatgtgggactgagaaatctgacaattgtggattctggattaaaatttgtggctcataaagcatttctgaaaaacagcaacctgcagcacatcaattttacccgaaacaaactgacgagtttgtctaggaaacatttccgtcaccttgacttgtctgaactgatcctggtgggcaatccatttacatgctcctgtgacattatgtggatcaagactctccaagaggctaaatccagtccagacactcaggatttgtactgcctgaatgaaagcagcaagaatattcccctggcaaacctgcagatacccaattgtggtttgccatctgcaaatctggccgcacctaacctcactgtggaggaaggaaagtctatcacattatcctgtagtgtggcaggtgatccggttcctaatatgtattgggatgttggtaacctggtttccaaacatatgaatgaaacaagccacacacagggctccttaaggataactaacatttcatccgatgacagtgggaagcagatctcttgtgtggcggaaaatcttgtaggagaagatcaagattctgtcaacctcactgtgcattttgcaccaactatcacatttctcgaatctccaacctcagaccaccactggtgcattccattcactgtgaaaggcaaccccaaaccagcgcttcagtggttctataacggggcaatattgaatgagtccaaatacatctgtactaaaatacatgttaccaatcacacggagtaccacggctgcctccagctggataatcccactcacatgaacaatggggactacactctaatagccaagaatgagtatgggaaggatgagaaacagatttctgctcacttcatgggctggcctggaattgacgatggtgcaaacccaaattatcctgatgtaatttatgaagattatggaactgcagcgaatgacatcggggacaccacgaacagaagtaatgaaatcccttccacagacgtcactgataaaaccggtcgggaacat

SEQ ID NO: 73 - DNA, 72 bp, Homo sapiens
ctctcggtctatgctgtggtggtgattgcgtctgtggtgggattttgccttttggtaatgctgtttctgctt

SEQ ID NO: 74 - DNA, 1152 bp, Homo sapiens
aagttggcaagacactccaagtttggcatgaaagatttctcatggtttggatttgggaaagtaaaatcaagacaaggtgttggcccagcctccgttatcagcaatgatgatgactctgccagcccactccatcacatctccaatgggagtaacactccatcttcttcggaaggtggcccagatgctgtcattattggaatgaccaagatccctgtcattgaaaatccccagtactttggcatcaccaacagtcagctcaagccagacacatttgttcagcacatcaagcgacataacattgttctgaaaagggagctaggcgaaggagcctttggaaaagtgttcctagctgaatgctataacctctgtcctgagcaggacaagatcttggtggcagtgaagaccctgaaggatgccagtgacaatgcacgcaaggacttccaccgtgaggccgagctcctgaccaacctccagcatgagcacatcgtcaagttctatggcgtctgcgtggagggcgaccccctcatcatggtctttgagtacatgaagcatggggacctcaacaagttcctcagggcacacggccctgatgccgtgctgatggctgagggcaacccgcccacggaactgacgcagtcgcagatgctgcatatagcccagcagatcgccgcgggcatggtctacctggcgtcccagcacttcgtgcaccgcgatttggccaccaggaactgcctggtcggggagaacttgctggtgaaaatcggggactttgggatgtcccgggacgtgtacagcactgactactacagggtcggtggccacacaatgctgcccattcgctggatgcctccagagagcatcatgtacaggaaattcacgacggaaagcgacgtctggagcctgggggtcgtgttgtgggagattttcacctatggcaaacagccctggtaccagctgtcaaacaatgaggtgatagagtgtatcactcagggccgagtcctgcagcgaccccgcacgtgcccccaggaggtgtatgagctgatgctggggtgctggcagcgagagccccacatgaggaagaacatcaagggcatccataccctccttcagaacttggccaaggcatctccggtctacctggacattctaggc

SEQ ID NO: 75 - protein, 822 aa, Homo sapiens
  MISC_FEATURE (1)..(31): Signal Peptide
  MISC_FEATURE (32)..(430): Extracellular Domain
  MISC_FEATURE (431)..(454): Transmembrane Domain
  MISC_FEATURE (455)..(822): Cytoplasmic Domain
MSSWIRWHGPAMARLWGFCWLVVGFWRAAFACPTSCKCSASRIWCSDPSPGIVAFPRLEPNSVDPENITEIFIANQKRLEIINEDDVEAYVGLRNLTIVDSGLKFVAHKAFLKNSNLQHINFTRNKLTSLSRKHFRHLDLSELILVGNPFTCSCDIMWIKTLQEAKSSPDTQDLYCLNESSKNIPLANLQIPNCGLPSANLAAPNLTVEEGKSITLSCSVAGDPVPNMYWDVGNLVSKHMNETSHTQGSLRITNISSDDSGKQISCVAENLVGEDQDSVNLTVHFAPTITFLESPTSDHHWCIPFTVKGNPKPALQWFYNGAILNESKYICTKIHVTNHTEYHGCLQLDNPTHMNNGDYTLIAKNEYGKDEKQISAHFMGWPGIDDGANPNYPDVIYEDYGTAANDIGDTTNRSNEIPSTDVTDKTGREHLSVYAVVVIASVVGFCLLVMLFLLKLARHSKFGMKGPASVISNDDDSASPLHHISNGSNTPSSSEGGPDAVIIGMTKIPVIENPQYFGITNSQLKPDTFVQHIKRHNIVLKRELGEGAFGKVFLAECYNLCPEQDKILVAVKTLKDASDNARKDFHREAELLTNLQHEHIVKFYGVCVEGDPLIMVFEYMKHGDLNKFLRAHGPDAVLMAEGNPPTELTQSQMLHIAQQIAAGMVYLASQHFVHRDLATRNCLVGENLLVKIGDFGMSRDVYSTDYYRVGGHTMLPIRWMPPESIMYRKFTTESDVWSLGVVLWEIFTYGKQPWYQLSNNEVIECITQGRVLQRPRTCPQEVYELMLGCWQREPHMRKNIKGIHTLLQNLAKASPVYLDILG

SEQ ID NO: 76 - DNA, 8498 bp, Homo sapiens
cctcgaggtgcataccggacccccattcgcatctaacaaggaatctgcgccccagagagtcccgggagcgccgccggtcggtgcccggcgcgccgggccatgcagcgacggccgccgcggagctccgagcagcggtagcgcccccctgtaaagcggttcgctatgccggggccactgtgaaccctgccgcctgccggaacactcttcgctccggaccagctcagcctctgataagctggactcggcacgcccgcaacaagcaccgaggagttaagagagccgcaagcgcagggaaggcctccccgcacgggtgggggaaagcggccggtgcagcgcggggacaggcactcgggctggcactggctgctagggatgtcgtcctggataaggtggcatggacccgccatggcgcggctctggggcttctgctggctggttgtgggcttctggagggccgctttcgcctgtcccacgtcctgcaaatgcagtgcctctcggatctggtgcagcgacccttctcctggcatcgtggcatttccgagattggagcctaacagtgtagatcctgagaacatcaccgaaattttcatcgcaaaccagaaaaggttagaaatcatcaacgaagatgatgttgaagcttatgtgggactgagaaatctgacaattgtggattctggattaaaatttgtggctcataaagcatttctgaaaaacagcaacctgcagcacatcaattttacccgaaacaaactgacgagtttgtctaggaaacatttccgtcaccttgacttgtctgaactgatcctggtgggcaatccatttacatgctcctgtgacattatgtggatcaagactctccaagaggctaaatccagtccagacactcaggatttgtactgcctgaatgaaagcagcaagaatattcccctggcaaacctgcagatacccaattgtggtttgccatctgcaaatctggccgcacctaacctcactgtggaggaaggaaagtctatcacattatcctgtagtgtggcaggtgatccggttcctaatatgtattgggatgttggtaacctggtttccaaacatatgaatgaaacaagccacacacagggctccttaaggataactaacatttcatccgatgacagtgggaagcagatctcttgtgtggcggaaaatcttgtaggagaagatcaagattctgtcaacctcactgtgcattttgcaccaactatcacatttctcgaatctccaacctcagaccaccactggtgcattccattcactgtgaaaggcaaccccaaaccagcgcttcagtggttctataacggggcaatattgaatgagtccaaatacatctgtactaaaatacatgttaccaatcacacggagtaccacggctgcctccagctggataatcccactcacatgaacaatggggactacactctaatagccaagaatgagtatgggaaggatgagaaacagatttctgctcacttcatgggctggcctggaattgacgatggtgcaaacccaaattatcctgatgtaatttatgaagattatggaactgcagcgaatgacatcggggacaccacgaacagaagtaatgaaatcccttccacagacgtcactgataaaaccggtcgggaacatctctcggtctatgctgtggtggtgattgcgtctgtggtgggattttgccttttggtaatgctgtttctgcttaagttggcaagacactccaagtttggcatgaaaggcccagcctccgttatcagcaatgatgatgactctgccagcccactccatcacatctccaatgggagtaacactccatcttcttcggaaggtggcccagatgctgtcattattggaatgaccaagatccctgtcattgaaaatccccagtactttggcatcaccaacagtcagctcaagccagacacatttgttcagcacatcaagcgacataacattgttctgaaaagggagctaggcgaaggagcctttggaaaagtgttcctagctgaatgctataacctctgtcctgagcaggacaagatcttggtggcagtgaagaccctgaaggatgccagtgacaatgcacgcaaggacttccaccgtgaggccgagctcctgaccaacctccagcatgagcacatcgtcaagttctatggcgtctgcgtggagggcgaccccctcatcatggtctttgagtacatgaagcatggggacctcaacaagttcctcagggcacacggccctgatgccgtgctgatggctgagggcaacccgcccacggaactgacgcagtcgcagatgctgcatatagcccagcagatcgccgcgggcatggtctacctggcgtcccagcacttcgtgcaccgcgatttggccaccaggaactgcctggtcggggagaacttgctggtgaaaatcggggactttgggatgtcccgggacgtgtacagcactgactactacagggtcggtggccacacaatgctgcccattcgctggatgcctccagagagcatcatgtacaggaaattcacgacggaaagcgacgtctggagcctgggggtcgtgttgtgggagattttcacctatggcaaacagccctggtaccagctgtcaaacaatgaggtgatagagtgtatcactcagggccgagtcctgcagcgaccccgcacgtgcccccaggaggtgtatgagctgatgctggggtgctggcagcgagagccccacatgaggaagaacatcaagggcatccataccctccttcagaacttggccaaggcatctccggtctacctggacattctaggctagggcccttttccccagaccgatccttcccaacgtactcctcagacgggctgagaggatgaacatcttttaactgccgctggaggccaccaagctgctctccttcactctgacagtattaacatcaaagactccgagaagctctcgagggaagcagtgtgtacttcttcatccatagacacagtattgacttctttttggcattatctctttctctctttccatctcccttggttgttcctttttctttttttaaattttctttttcttttttttttcgtcttccctgcttcacgattcttaccctttcttttgaatcaatctggcttctgcattactattaactctgcatagacaaaggccttaacaaacgtaatttgttatatcagcagacactccagtttgcccaccacaactaacaatgccttgttgtattcctgcctttgatgtggatgaaaaaaagggaaaacaaatatttcacttaaactttgtcacttctgctgtacagatatcgagagtttctatggattcacttctatttatttattattattactgttcttattgtttttggatggcttaagcctgtgtataaaaaagaaaacttgtgttcaatctgtgaagcctttatctatgggagattaaaaccagagagaaagaagatttattatgaaccgcaatatgggaggaacaaagacaaccactgggatcagctggtgtcagtccctacttaggaaatactcagcaactgttagctgggaagaatgtattcggcaccttcccctgaggacctttctgaggagtaaaaagactactggcctctgtgccatggatgattcttttcccatcaccagaaatgatagcgtgcagtagagagcaaagatggcttccgtgagacacaagatggcgcatagtgtgctcggacacagttttgtcttcgtaggttgtgatgatagcactggtttgtttctcaagcgctatccacagaacctttgtcaacttcagttgaaaagaggtggattcatgtccagagctcatttcggggtcaggtgggaaagccaagaacttggaaaagataagacaagctataaattcggaggcaagtttcttttacaatgaacttttcagatctcacttccctccgacccctaacttccatgcccacccgtccttttaactgtgcaagcaaaattgtgcatggtcttcgtcgattaataccttgtgtgcagacactactgctccagacgtcgtttccctgataggtagagcagatccataaaaaggtatgacttatacaattaggggaagctaatggagtttattagctgagtatcaatgtctctgcgttgtacggtggtgatgggttttaatgaatatggaccctgaagcctggaaatcctcatccacgtcgaacccacaggactgtgggaagggcagaatcaatccctaagggaaaggaaacctcaccctgagggcatcacatgcactcatgttcagtgtacacaggtcaagtcccttgctctgggctctagttgggagagtggtttcattccaagtgtactccattgtcagtatgctgtttttgtttccttcactccattcaaaaagtcaaaatacaaaatttggcacagcatgccaacgggaggctgtgcccagaccaagcactggaagtgtgcttctaggcatagtcattggttttgcaaaaagagggctcaaatttaaatagaaatttacagctatttgaatggtcagatataccaagaaagaaaaatatttctgttcctcaagaaaacttgctaccctctgtgaggggaattttgctaaacttgacatctttataacatgagccagattgaaagggagtgattttcattcatcttaggtcatgttatttcatatttgtttctgaaggtgcgatagctctgttttaggttttgcttgcgcctgttaattactggaacaccttatttttcattaaaggctttgaaagccaattctcaaaaattcaaaagtgcaaattaacagaacaaaaggaaatccagtagcaactgcagtcaagcgagggagttgacaagataaaccttacgtccattcaagttatatgctggcctatgagagatgagagttgggtcgtttgttctctttgttgatgattttaaaaaaaccctctagaatacacataataacataatgaaagccatatctccatgatatatatgtgcacatatatatacatacatgtgcatgtatgtatcatattaaggacccatggtactcttaaaacactgtagaactctgtgacgcagtaaggaaggggcagatttgtacaaaaacttttctagattccatcagcaaaaaccaacacaggtttgtcacgctgcatgtctggccagctaatctcgggggaaaagctacaagttatttattttattttaagagaataaagtaggtaataatttaagggatcaaattcaaggaggaatgtgcaattttagagcaaagatttgtttaaggcaaatgagactttgggagcatcccattccagttttgtcttttttttctctgaaagaaaaaagcaaaaaataaaataaaattccacttataccttctgacaagtccctaaaggtcttgaaataaaaggttctatgcaagtgcaaagttttatagttatttttattgctgattattactattactatctctgttgtcttaagagtatgtgctgatttcagagacatctcaaattgaaagaatatcagattgcttttaaagtagctgaacgagccacagaatatctgaaattattcattgttgttcctccaccaccccctttctcatggtctgatttttagaagagtggcatcctcgttctaaaatgtaatgatcaccaaatacggccttccatcaaatttgtgaaaactacaacagtataacagtgacaaacctaattctctagcccaaacctggtctgacaatcatttccatttagaagtcattgaatagttttccaaacactttccatgtgtgttagcaaattattcctattttgtgtagatgaggacgttgagactcagagacattcagaggcacgctagaggtctccagcctagcttccagcaccattgggactgaatccaagtactctcactctgaacttcgtggttctgtccactagagactctaatatgcaaacaagcagttcaggaaagaaagcatgctaacacattcatgaagcagtatatgaagttagaagaacaaaaggaaatacaggagatgacaagcaactgagatattgtgatatataatcatgctcttagcttcagctaaattcagctaaattcttgtacactgaaccaatgtcataatcaggcttatttagaaaacactttgaactatgctataaaagattatatcagaattcatattatacatgtgttcacatcagcgctacctgtgatgttttcatgtatttatgtatgtgttataaatacttgatttatacatatacaaatgcacatacgtagtgtgtttgtgtgtttatgtataaatttataggcacacaataatagaggtaattataagtaggatgcggtatgaataatttgcttaaaatatgctaaataaccaaaactgtttaacgtcatgttgctgttagtgcttccatactccacgtgggtaggactacatcacacttttcaactctgtgcagtactgcatgggtggaagacatatttaagataatgtgcttcccaaaacaactgaataaaagccatcccactacattgagtgctttctctggctccttgcaaagaaagatactttttgtaatggtccaggaaaggaacattgctttctttttgtctttcagcacatttgtattatgctcaccttgtctctgtctcactgtgacccctttacacttgagttcagagttcaagcattccaaatataaattggaatgttggcagcccagtggcttgaaggccaatgatgagcagtccaagaccccacagcgagatgagcaactcttaggaattcccacatcctagagtgaatgcaccaactaacagtatagaatgctgtccttttcaaagcgtcctaacagcaggattacctggtcaagtatggactttctttgaatctttcttttcacaaattggactgcctgtaataccaataacattgttgtatctaactaaataaatgactgcatatacacacataccctcaattctcttgcttccccattttctttttcatcccctgtctcaggacttttattttcaatgttgacctttggtttggccatatatcactgttataggaaatctcatgagaggaatggctagtgacccaactctccaaatgtctaagttagtagttacagctgattttttatgatgcataattggaatgtggagcctctgaggttgtgatagcttgtacatgaatttcaaatgtcattctaaagaatgaggggtgggagggatttatagttagaaacgacagtgcaggaaggggtattttcttgttgtcagggctggaatgaatcactgctgctcaagtcaaaggttcttgaatatccttagtttttgcatttcccctccttttcctttgacctttatttatttaattatgtatttatttatttatttatatacttttgctccattcagcacaaacacaaagcaaagcaaaaaaaaaaatatatatatatatatctgtatatgtgttgtaggcaaaacactgtgaatttcacaacaaccaccaccaagcaactattttgccatcttaacatacatctcaggagacgaaatgagaaaagatggggatgtcattttttagtctatgcgtttgaggccaggtccatgtttatttatttctttagtctatgcattaatgaaaatgatcctgagtggaggttagctgaacgttcaatgtactggagcaagcatcataaaagctgctagtagccatgtgtttgaacaggaaaaatattacagaaaatgaaatgtaaaggcctatatcttgcagcttgtatatcttactattgcttaaaaaatgtataaagcagctggaaatgttttaaatacaaggtctttgaattaaatgtggattttaaatatgtaatcccttgacaaatgaccaaattatggtgaactattgctccctgcgttctttgatcattacctatgacttacaaatctgcctggagatgtggacattctgcatttgcttctgtatctggagagatgtttgtatatatccaggccgtatacacacacatttccatatctctctacagatatatttccccttcaatcgtgacctggtatttggaactctccttttcatttggcttatcttccttttaatgtgatgtctctgtgctaatacttaccagttcttgttttgcaatctgttttgaggtccattgctttactaagacccactgcatcttggctgatttcaaagtgacacctgaatacagtgtttaaaaaaaaaaaagttttgtttgtaaatcatgtgaccagcttctctcaacctgacatggaaagtctcttgtactacagtgtatttaataaaaatgatgtcttacaataaataacatactccaaaagagagactaaaaatgaaaaaaaaaaaaaaaaaaaaaaaaa

SEQ ID NO: 77 - DNA, 2469 bp, Homo sapiens
  misc_feature (1)..(93): Signal Peptide
  misc_feature (94)..(1290): Extracellular Domain
  misc_feature (1291)..(1362): Transmembrane Domain
  misc_feature (1363)..(2466): Cytoplasmic Domain
atgtcgtcctggataaggtggcatggacccgccatggcgcggctctggggcttctgctggctggttgtgggcttctggagggccgctttcgcctgtcccacgtcctgcaaatgcagtgcctctcggatctggtgcagcgacccttctcctggcatcgtggcatttccgagattggagcctaacagtgtagatcctgagaacatcaccgaaattttcatcgcaaaccagaaaaggttagaaatcatcaacgaagatgatgttgaagcttatgtgggactgagaaatctgacaattgtggattctggattaaaatttgtggctcataaagcatttctgaaaaacagcaacctgcagcacatcaattttacccgaaacaaactgacgagtttgtctaggaaacatttccgtcaccttgacttgtctgaactgatcctggtgggcaatccatttacatgctcctgtgacattatgtggatcaagactctccaagaggctaaatccagtccagacactcaggatttgtactgcctgaatgaaagcagcaagaatattcccctggcaaacctgcagatacccaattgtggtttgccatctgcaaatctggccgcacctaacctcactgtggaggaaggaaagtctatcacattatcctgtagtgtggcaggtgatccggttcctaatatgtattgggatgttggtaacctggtttccaaacatatgaatgaaacaagccacacacagggctccttaaggataactaacatttcatccgatgacagtgggaagcagatctcttgtgtggcggaaaatcttgtaggagaagatcaagattctgtcaacctcactgtgcattttgcaccaactatcacatttctcgaatctccaacctcagaccaccactggtgcattccattcactgtgaaaggcaaccccaaaccagcgcttcagtggttctataacggggcaatattgaatgagtccaaatacatctgtactaaaatacatgttaccaatcacacggagtaccacggctgcctccagctggataatcccactcacatgaacaatggggactacactctaatagccaagaatgagtatgggaaggatgagaaacagatttctgctcacttcatgggctggcctggaattgacgatggtgcaaacccaaattatcctgatgtaatttatgaagattatggaactgcagcgaatgacatcggggacaccacgaacagaagtaatgaaatcccttccacagacgtcactgataaaaccggtcgggaacatctctcggtctatgctgtggtggtgattgcgtctgtggtgggattttgccttttggtaatgctgtttctgcttaagttggcaagacactccaagtttggcatgaaaggcccagcctccgttatcagcaatgatgatgactctgccagcccactccatcacatctccaatgggagtaacactccatcttcttcggaaggtggcccagatgctgtcattattggaatgaccaagatccctgtcattgaaaatccccagtactttggcatcaccaacagtcagctcaagccagacacatttgttcagcacatcaagcgacataacattgttctgaaaagggagctaggcgaaggagcctttggaaaagtgttcctagctgaatgctataacctctgtcctgagcaggacaagatcttggtggcagtgaagaccctgaaggatgccagtgacaatgcacgcaaggacttccaccgtgaggccgagctcctgaccaacctccagcatgagcacatcgtcaagttctatggcgtctgcgtggagggcgaccccctcatcatggtctttgagtacatgaagcatggggacctcaacaagttcctcagggcacacggccctgatgccgtgctgatggctgagggcaacccgcccacggaactgacgcagtcgcagatgctgcatatagcccagcagatcgccgcgggcatggtctacctggcgtcccagcacttcgtgcaccgcgatttggccaccaggaactgcctggtcggggagaacttgctggtgaaaatcggggactttgggatgtcccgggacgtgtacagcactgactactacagggtcggtggccacacaatgctgcccattcgctggatgcctccagagagcatcatgtacaggaaattcacgacggaaagcgacgtctggagcctgggggtcgtgttgtgggagattttcacctatggcaaacagccctggtaccagctgtcaaacaatgaggtgatagagtgtatcactcagggccgagtcctgcagcgaccccgcacgtgcccccaggaggtgtatgagctgatgctggggtgctggcagcgagagccccacatgaggaagaacatcaagggcatccataccctccttcagaacttggccaaggcatctccggtctacctggacattctaggctag

SEQ ID NO: 78 - DNA, 354 bp, Artificial Sequence
  Synthetic
caggtgcagctggtggagtctgggggaggcgtggtccagcctgggaggtccctgagactctcctgtgcagcctctggattcagcttcagtagctttggcatgcactgggtccgccaggctccaggcaagggactggagtgggtgtcagttatatcatatgatggaattaatacatactatacagactccgtgaagggccgattcaccatctccagagacaattccaagaacacgctgtatctgcaaatgaacggcctgagagctgaggacacggctctttattactgtgtgcaagggtcaattggaaccgtttttgaatactggggccagggaaccctggtcaccgtctcctca

SEQ ID NO: 79 - protein, 118 aa, Artificial Sequence
  Synthetic
QVQLVESGGGVVQPGRSLRLSCAASGFSFSSFGMHWVRQAPGKGLEWVSVISYDGINTYYTDSVKGRFTISRDNSKNTLYLQMNGLRAEDTALYYCVQGSIGTVFEYWGQGTLVTVSS

SEQ ID NO: 80 - DNA, 24 bp, Artificial Sequence
  Synthetic
ggattcagcttcagtagctttggc

SEQ ID NO: 81 - protein, 8 aa, Artificial Sequence
  Synthetic
GFSFSSFG

SEQ ID NO: 82 - DNA, 24 bp, Artificial Sequence
  Synthetic
atatcatatgatggaattaataca

SEQ ID NO: 83 - protein, 8 aa, Artificial Sequence
  Synthetic
ISYDGINT

SEQ ID NO: 84 - DNA, 33 bp, Artificial Sequence
  Synthetic
gtgcaagggtcaattggaaccgtttttgaatac

SEQ ID NO: 85 - protein, 11 aa, Artificial Sequence
  Synthetic
VQGSIGTVFEY

SEQ ID NO: 86 - DNA, 321 bp, Artificial Sequence
  Synthetic
gacatccagatgacccagtctccatcctccctgtctgcatctgtaggagacagagtcaccatcacttgccgggcgagtcagggcattagcaattatttagcctggtatcagcagaaaccagggaaagttcctaaactcctgatctatgctgcatccactttacaatcaggggtcccatctcggttcggtggcagtggatctgggacagatttcactctcaccatcagcagcctgcagcctgaagatgttgcaacttattactgtcaaaagtataccagtgccccattcactttcggccctgggaccaaagtggatatcaaa

SEQ ID NO: 87 - protein, 107 aa, Artificial Sequence
  Synthetic
DIQMTQSPSSLSASVGDRVTITCRASQGISNYLAWYQQKPGKVPKLLIYAASTLQSGVPSRFGGSGSGTDFTLTISSLQPEDVATYYCQKYTSAPFTFGPGTKVDIK

SEQ ID NO: 88 - DNA, 18 bp, Artificial Sequence
  Synthetic
cagggcattagcaattat

SEQ ID NO: 89 - protein, 6 aa, Artificial Sequence
  Synthetic
QGISNY

SEQ ID NO: 90 - DNA, 9 bp, Artificial Sequence
  Synthetic
gctgcatcc

SEQ ID NO: 91 - protein, 3 aa, Artificial Sequence
  Synthetic
AAS

SEQ ID NO: 92 - DNA, 27 bp, Artificial Sequence
  Synthetic
caaaagtataccagtgccccattcact

SEQ ID NO: 93 - protein, 9 aa, Artificial Sequence
  Synthetic
QKYTSAPFT

SEQ ID NO: 94 - DNA, 366 bp, Artificial Sequence
  Synthetic
gaggtgcagctggtggagtctgggggaggcttggtccagcctggggggtccctaaaactctcctgtacagcctctgggttcaccttcagtggctctgttattcactgggtccgccaggcttccgggaaagggctggagtggattggccgtattagaaacaaggctaacagttacgcgacagcatatggtgcgtcggtgacaggcaggttcaccatctccagagatgattcaaagaacacggcgtatctgcaaatgaacagcctgaaaaccgaggacacggccgtttattactgtactttcccgggtgtagtgggacgaggaggttttgactactggggccagggcaccctggtcaccgtctcctca

SEQ ID NO: 95 - protein, 122 aa, Artificial Sequence
  Synthetic
EVQLVESGGGLVQPGGSLKLSCTASGFTFSGSVIHWVRQASGKGLEWIGRIRNKANSYATAYGASVTGRFTISRDDSKNTAYLQMNSLKTEDTAVYYCTFPGVVGRGGFDYWGQGTLVTVSS

SEQ ID NO: 96 - DNA, 24 bp, Artificial Sequence
  Synthetic
gggttcaccttcagtggctctgtt

SEQ ID NO: 97 - protein, 8 aa, Artificial Sequence
  Synthetic
GFTFSGSV

SEQ ID NO: 98 - DNA, 30 bp, Artificial Sequence
  Synthetic
attagaaacaaggctaacagttacgcgaca

SEQ ID NO: 99 - protein, 10 aa, Artificial Sequence
  Synthetic
IRNKANSYAT

SEQ ID NO: 100 - DNA, 39 bp, Artificial Sequence
  Synthetic
actttcccgggtgtagtgggacgaggaggttttgactac

SEQ ID NO: 101 - protein, 13 aa, Artificial Sequence
  Synthetic
TFPGVVGRGGFDY

SEQ ID NO: 102 - DNA, 339 bp, Artificial Sequence
  Synthetic
gacatcgtgatgacccagtctccagactccctggctgtgtctctgggcgagggggccaccatcaactgcatgtccagccagagtgttttattcagctccaacaataagaactacttagcttggtaccaacagaaaccaggacagcctcctaagttgctcttttactgggcatctacccgggaatccggggtccctgaccgattcggtggcagcgggtctgggacagatttctctctcaccatcaacagcctgcagactgaagatgtggcagtttattactgtctccaatattatagtattccgtggacgttcggccaagggaccaaggtggaaatcaaa

SEQ ID NO: 103 - protein, 113 aa, Artificial Sequence
  Synthetic
DIVMTQSPDSLAVSLGEGATINCMSSQSVLFSSNNKNYLAWYQQKPGQPPKLLFYWASTRESGVPDRFGGSGSGTDFSLTINSLQTEDVAVYYCLQYYSIPWTFGQGTKVEIK

SEQ ID NO: 104 - DNA, 36 bp, Artificial Sequence
  Synthetic
cagagtgttttattcagctccaacaataagaactac

SEQ ID NO: 105 - protein, 12 aa, Artificial Sequence
  Synthetic
QSVLFSSNNKNY

SEQ ID NO: 106 - DNA, 9 bp, Artificial Sequence
  Synthetic
tgggcatct

SEQ ID NO: 107 - protein, 3 aa, Artificial Sequence
  Synthetic
WAS

SEQ ID NO: 108 - DNA, 27 bp, Artificial Sequence
  Synthetic
ctccaatattatagtattccgtggacg

SEQ ID NO: 109 - protein, 9 aa, Artificial Sequence
  Synthetic
LQYYSIPWT

SEQ ID NO: 110 - DNA, 381 bp, Artificial Sequence
  Synthetic
gaggtgcagctggtggagtctgggggaggcttggtacagcctggagggtccctgacactctcctgtgcagcctctggattcaatttccgtgattatgaaatgatctgggtccgccagactccagggaaggggctggagtggatttcatacattagtaatagtggttataccatatactacgcagactctgtgaagggccgattcaccatctccagagacaacgccaggaactcaatatatctgcaagtgaacagcctgagagccgaggacacggctgtttattactgttcgagacgtactactatgattcggggcattagggcgtactactattacggtctggacgtctggggccaagggaccacggtcaccgtctcctca

SEQ ID NO: 111 - protein, 127 aa, Artificial Sequence
  Synthetic
EVQLVESGGGLVQPGGSLTLSCAASGFNFRDYEMIWVRQTPGKGLEWISYISNSGYTIYYADSVKGRFTISRDNARNSIYLQVNSLRAEDTAVYYCSRRTTMIRGIRAYYYYGLDVWGQGTTVTVSS

SEQ ID NO: 112 - DNA, 24 bp, Artificial Sequence
  Synthetic
ggattcaatttccgtgattatgaa

SEQ ID NO: 113 - protein, 8 aa, Artificial Sequence
  Synthetic
GFNFRDYE

SEQ ID NO: 114 - DNA, 24 bp, Artificial Sequence
  Synthetic
attagtaatagtggttataccata

SEQ ID NO: 115 - protein, 8 aa, Artificial Sequence
  Synthetic
ISNSGYTI

SEQ ID NO: 116 - DNA, 60 bp, Artificial Sequence
  Synthetic
tcgagacgtactactatgattcggggcattagggcgtactactattacggtctggacgtc

SEQ ID NO: 117 - protein, 20 aa, Artificial Sequence
  Synthetic
SRRTTMIRGIRAYYYYGLDV

SEQ ID NO: 118 - DNA, 324 bp, Artificial Sequence
  Synthetic
gacatccagatgacccagtctccatcctccctgtctgcatctgtaggagacagagtcaccatcacttgccgggcaagtcagagcattagcagctatttaaattggtatcagcagaaaccagggaaagcccctaagctcctgatctatgctgcatccagtttgcaaagtggggtcccgtcaaggttcagtggcagtggatctgggacagatttcactctcaccatcagcagtctgcaacctgaagattttgcaacttactactgtcaacagagttacagtacccctccgatcaccttcggccaagggacacgactggagattaaa

SEQ ID NO: 119 - protein, 108 aa, Artificial Sequence
  Synthetic
DIQMTQSPSSLSASVGDRVTITCRASQSISSYLNWYQQKPGKAPKLLIYAASSLQSGVPSRFSGSGSGTDFTLTISSLQPEDFATYYCQQSYSTPPITFGQGTRLEIK

SEQ ID NO: 120 - DNA, 18 bp, Artificial Sequence
  Synthetic
cagagcattagcagctat

SEQ ID NO: 121 - protein, 6 aa, Artificial Sequence
  Synthetic
QSISSY

SEQ ID NO: 122 - DNA, 9 bp, Artificial Sequence
  Synthetic
gctgcatcc

SEQ ID NO: 123 - protein, 3 aa, Artificial Sequence
  Synthetic
AAS

SEQ ID NO: 124 - DNA, 30 bp, Artificial Sequence
  Synthetic
caacagagttacagtacccctccgatcacc

SEQ ID NO: 125 - protein, 10 aa, Artificial Sequence
  Synthetic
QQSYSTPPIT